European Patent Specification EP 3 619 539 B1, published February 14, 2024. Title: METHOD. Applicant: OXFORD NANOPORE TECHNOLOGIES LIMITED. The sequence listing filed with the application follows.

SEQUENCE LISTING (64 sequences)

SEQ ID NO: 1 - DNA, 1863 bp, Artificial Sequence
  Synthetic reporter polynucleotide
  misc_feature (1)..(1): 5' Biotinylation
attgcuacttgcctgtcgctctatcttctggtgctgaagaaagttgtcggtgtctttgtgttaacctacttgcctgtcgctctatcttcggcgtctgcttgggtgtttaaccgtctctcttgtccgtgcaatagctcaataatagaataaaacgatcaatatctattttatcgatcgtttatatcgatcgataagctaataataacctttgtcagtaacatgcacagatacgtacagaaagacattcagggaacaacagaaccacaattcagaaactcccacagccggacctccggcactgtaaccctttacctgccggtatccacgtttgtgggtaccggcttttttattcaccctcaatctaaggaaaagctgatgaaacgacatctgaatacctgctacaggctggtatggaatcacatgacgggcgctttcgtggttgcctccgaactggcccgcgcacggggtaaacgtggcggtgtggcggttgcactgtctcttgccgcagtcacgtcactcccggtgctggctgctgacatcgttgtgcacccgggagaaaccgtgaacggcggaacactggcaaatcatgacaaccagattgtcttcggtacgaccaacggaatgaccatcagtaccgggctggagtatgggccggataacgaggccaataccggcgggcaatgggtacaggatggcggaacagccaacaaaacgactgtcaccagtggtggtcttcagagagtgaaccccggtggaagtgtctcagacacggttatcagtgccggaggcggacagagccttcagggacgggctgtgaacaccacgctgaatggtggcgaacagtggatgcatgagggggcgatagccacaggaaccgtcattaatgataagggctggcaggtcgtcaagcccggtacagtggcaacggataccgttgttaataccggggcggaagggggaccggatgcagaaaacggtgataccgggcagtttgttcgcggggatgccgtacgcacaaccatcaataaaaacggtcgccagattgtgagagctgaaggaacggcaaataccactgtggtttatgccggcggcgaccagactgtacatggtcacgcactggataccacgctgaatgggggataccagtatgtgcacaacggcggtacagcgtctgacactgttgtgaacagtgacggctggcagattgtcaaaaacgggggtgtggccgggaataccaccgttaatcagaagggcagactgcaggtggacgccggtggtacagccacgaatgtcaccctgaagcagggcggcgcactggttaccagtacggctgcaaccgttaccggcataaaccgcctgggagcattctctgttgtggagggtaaagctgataatgtcgtactggaaaatggcggacgcctggatgtgctgaccggacacacagccactaatacccgcgtggatgatggcggaacgctggatgtccgcaacggtggcaccgccaccaccgtatccatgggaaatggcggtgtactgctggccgattccggtgccgctgtcagtggtacccggagcgacggaaaggcattcagtatcggaggcggtcaggcggatgccctgatgctggaaaaaggcagttcattcacgctgaacgccggtgatacggccacggataccacggtaaatggcggactgttcaccgccaggggcggcacactggcgggcaccaccacgctgaataacggcgccaaaggttaaacacccaagcagacgccgcaatatcagcaccaacagaaaggttaacacaaagacaccgacaactttcttcagcaccagaagatagagcgacaggcaagtagcaat

SEQ ID NO: 2 - DNA, 1863 bp, Artificial Sequence
  Synthetic reporter polynucleotide
  misc_feature (1)..(1): 5' Biotinylation
attgcuacttgcctgtcgctctatcttctggtgctgtcgattccgtttgtagtcgtctgtttaacctacttgcctgtcgctctatcttcggcgtctgcttgggtgtttaaccgtctctcttgtccgtgcaatagctcaataatagaataaaacgatcaatatctattttatcgatcgtttatatcgatcgataagctaataataacctttgtcagtaacatgcacagatacgtacagaaagacattcagggaacaacagaaccacaattcagaaactcccacagccggacctccggcactgtaaccctttacctgccggtatccacgtttgtgggtaccggcttttttattcaccctcaatctaaggaaaagctgatgaaacgacatctgaatacctgctacaggctggtatggaatcacatgacgggcgctttcgtggttgcctccgaactggcccgcgcacggggtaaacgtggcggtgtggcggttgcactgtctcttgccgcagtcacgtcactcccggtgctggctgctgacatcgttgtgcacccgggagaaaccgtgaacggcggaacactggcaaatcatgacaaccagattgtcttcggtacgaccaacggaatgaccatcagtaccgggctggagtatgggccggataacgaggccaataccggcgggcaatgggtacaggatggcggaacagccaacaaaacgactgtcaccagtggtggtcttcagagagtgaaccccggtggaagtgtctcagacacggttatcagtgccggaggcggacagagccttcagggacgggctgtgaacaccacgctgaatggtggcgaacagtggatgcatgagggggcgatagccacaggaaccgtcattaatgataagggctggcaggtcgtcaagcccggtacagtggcaacggataccgttgttaataccggggcggaagggggaccggatgcagaaaacggtgataccgggcagtttgttcgcggggatgccgtacgcacaaccatcaataaaaacggtcgccagattgtgagagctgaaggaacggcaaataccactgtggtttatgccggcggcgaccagactgtacatggtcacgcactggataccacgctgaatgggggataccagtatgtgcacaacggcggtacagcgtctgacactgttgtgaacagtgacggctggcagattgtcaaaaacgggggtgtggccgggaataccaccgttaatcagaagggcagactgcaggtggacgccggtggtacagccacgaatgtcaccctgaagcagggcggcgcactggttaccagtacggctgcaaccgttaccggcataaaccgcctgggagcattctctgttgtggagggtaaagctgataatgtcgtactggaaaatggcggacgcctggatgtgctgaccggacacacagccactaatacccgcgtggatgatggcggaacgctggatgtccgcaacggtggcaccgccaccaccgtatccatgggaaatggcggtgtactgctggccgattccggtgccgctgtcagtggtacccggagcgacggaaaggcattcagtatcggaggcggtcaggcggatgccctgatgctggaaaaaggcagttcattcacgctgaacgccggtgatacggccacggataccacggtaaatggcggactgttcaccgccaggggcggcacactggcgggcaccaccacgctgaataacggcgccaaaggttaaacacccaagcagacgccgcaatatcagcaccaacagaaaggttaaacagacgactacaaacggaatcgacagcaccagaagatagagcgacaggcaagtagcaat

SEQ ID NO: 3 - DNA, 1863 bp, Artificial Sequence
  Synthetic reporter polynucleotide
  misc_feature (1)..(1): 5' Biotinylation
attgcuacttgcctgtcgctctatcttctggtgctggagtcttgtgtcccagttaccaggttaacctacttgcctgtcgctctatcttcggcgtctgcttgggtgtttaaccgtctctcttgtccgtgcaatagctcaataatagaataaaacgatcaatatctattttatcgatcgtttatatcgatcgataagctaataataacctttgtcagtaacatgcacagatacgtacagaaagacattcagggaacaacagaaccacaattcagaaactcccacagccggacctccggcactgtaaccctttacctgccggtatccacgtttgtgggtaccggcttttttattcaccctcaatctaaggaaaagctgatgaaacgacatctgaatacctgctacaggctggtatggaatcacatgacgggcgctttcgtggttgcctccgaactggcccgcgcacggggtaaacgtggcggtgtggcggttgcactgtctcttgccgcagtcacgtcactcccggtgctggctgctgacatcgttgtgcacccgggagaaaccgtgaacggcggaacactggcaaatcatgacaaccagattgtcttcggtacgaccaacggaatgaccatcagtaccgggctggagtatgggccggataacgaggccaataccggcgggcaatgggtacaggatggcggaacagccaacaaaacgactgtcaccagtggtggtcttcagagagtgaaccccggtggaagtgtctcagacacggttatcagtgccggaggcggacagagccttcagggacgggctgtgaacaccacgctgaatggtggcgaacagtggatgcatgagggggcgatagccacaggaaccgtcattaatgataagggctggcaggtcgtcaagcccggtacagtggcaacggataccgttgttaataccggggcggaagggggaccggatgcagaaaacggtgataccgggcagtttgttcgcggggatgccgtacgcacaaccatcaataaaaacggtcgccagattgtgagagctgaaggaacggcaaataccactgtggtttatgccggcggcgaccagactgtacatggtcacgcactggataccacgctgaatgggggataccagtatgtgcacaacggcggtacagcgtctgacactgttgtgaacagtgacggctggcagattgtcaaaaacgggggtgtggccgggaataccaccgttaatcagaagggcagactgcaggtggacgccggtggtacagccacgaatgtcaccctgaagcagggcggcgcactggttaccagtacggctgcaaccgttaccggcataaaccgcctgggagcattctctgttgtggagggtaaagctgataatgtcgtactggaaaatggcggacgcctggatgtgctgaccggacacacagccactaatacccgcgtggatgatggcggaacgctggatgtccgcaacggtggcaccgccaccaccgtatccatgggaaatggcggtgtactgctggccgattccggtgccgctgtcagtggtacccggagcgacggaaaggcattcagtatcggaggcggtcaggcggatgccctgatgctggaaaaaggcagttcattcacgctgaacgccggtgatacggccacggataccacggtaaatggcggactgttcaccgccaggggcggcacactggcgggcaccaccacgctgaataacggcgccaaaggttaaacacccaagcagacgccgcaatatcagcaccaacagaaaggttaacctggtaactgggacacaagactccagcaccagaagatagagcgacaggcaagtagcaat

SEQ ID NO: 4 - DNA, 1863 bp, Artificial Sequence
  Synthetic reporter polynucleotide
  misc_feature (1)..(1): 5' Biotinylation
attgcuacttgcctgtcgctctatcttctggtgctgcttgtccagggtttgtgtaaccttttaacctacttgcctgtcgctctatcttcggcgtctgcttgggtgtttaaccgtctctcttgtccgtgcaatagctcaataatagaataaaacgatcaatatctattttatcgatcgtttatatcgatcgataagctaataataacctttgtcagtaacatgcacagatacgtacagaaagacattcagggaacaacagaaccacaattcagaaactcccacagccggacctccggcactgtaaccctttacctgccggtatccacgtttgtgggtaccggcttttttattcaccctcaatctaaggaaaagctgatgaaacgacatctgaatacctgctacaggctggtatggaatcacatgacgggcgctttcgtggttgcctccgaactggcccgcgcacggggtaaacgtggcggtgtggcggttgcactgtctcttgccgcagtcacgtcactcccggtgctggctgctgacatcgttgtgcacccgggagaaaccgtgaacggcggaacactggcaaatcatgacaaccagattgtcttcggtacgaccaacggaatgaccatcagtaccgggctggagtatgggccggataacgaggccaataccggcgggcaatgggtacaggatggcggaacagccaacaaaacgactgtcaccagtggtggtcttcagagagtgaaccccggtggaagtgtctcagacacggttatcagtgccggaggcggacagagccttcagggacgggctgtgaacaccacgctgaatggtggcgaacagtggatgcatgagggggcgatagccacaggaaccgtcattaatgataagggctggcaggtcgtcaagcccggtacagtggcaacggataccgttgttaataccggggcggaagggggaccggatgcagaaaacggtgataccgggcagtttgttcgcggggatgccgtacgcacaaccatcaataaaaacggtcgccagattgtgagagctgaaggaacggcaaataccactgtggtttatgccggcggcgaccagactgtacatggtcacgcactggataccacgctgaatgggggataccagtatgtgcacaacggcggtacagcgtctgacactgttgtgaacagtgacggctggcagattgtcaaaaacgggggtgtggccgggaataccaccgttaatcagaagggcagactgcaggtggacgccggtggtacagccacgaatgtcaccctgaagcagggcggcgcactggttaccagtacggctgcaaccgttaccggcataaaccgcctgggagcattctctgttgtggagggtaaagctgataatgtcgtactggaaaatggcggacgcctggatgtgctgaccggacacacagccactaatacccgcgtggatgatggcggaacgctggatgtccgcaacggtggcaccgccaccaccgtatccatgggaaatggcggtgtactgctggccgattccggtgccgctgtcagtggtacccggagcgacggaaaggcattcagtatcggaggcggtcaggcggatgccctgatgctggaaaaaggcagttcattcacgctgaacgccggtgatacggccacggataccacggtaaatggcggactgttcaccgccaggggcggcacactggcgggcaccaccacgctgaataacggcgccaaaggttaaacacccaagcagacgccgcaatatcagcaccaacagaaaggttaaaaggttacacaaaccctggacaagcagcaccagaagatagagcgacaggcaagtagcaat

SEQ ID NO: 5 - DNA, 1863 bp, Artificial Sequence
  Synthetic reporter polynucleotide
  misc_feature (1)..(1): 5' Biotinylation
attgcuacttgcctgtcgctctatcttctggtgctgttctcgcaaaggcagaaagtagtcttaacctacttgcctgtcgctctatcttcggcgtctgcttgggtgtttaaccgtctctcttgtccgtgcaatagctcaataatagaataaaacgatcaatatctattttatcgatcgtttatatcgatcgataagctaataataacctttgtcagtaacatgcacagatacgtacagaaagacattcagggaacaacagaaccacaattcagaaactcccacagccggacctccggcactgtaaccctttacctgccggtatccacgtttgtgggtaccggcttttttattcaccctcaatctaaggaaaagctgatgaaacgacatctgaatacctgctacaggctggtatggaatcacatgacgggcgctttcgtggttgcctccgaactggcccgcgcacggggtaaacgtggcggtgtggcggttgcactgtctcttgccgcagtcacgtcactcccggtgctggctgctgacatcgttgtgcacccgggagaaaccgtgaacggcggaacactggcaaatcatgacaaccagattgtcttcggtacgaccaacggaatgaccatcagtaccgggctggagtatgggccggataacgaggccaataccggcgggcaatgggtacaggatggcggaacagccaacaaaacgactgtcaccagtggtggtcttcagagagtgaaccccggtggaagtgtctcagacacggttatcagtgccggaggcggacagagccttcagggacgggctgtgaacaccacgctgaatggtggcgaacagtggatgcatgagggggcgatagccacaggaaccgtcattaatgataagggctggcaggtcgtcaagcccggtacagtggcaacggataccgttgttaataccggggcggaagggggaccggatgcagaaaacggtgataccgggcagtttgttcgcggggatgccgtacgcacaaccatcaataaaaacggtcgccagattgtgagagctgaaggaacggcaaataccactgtggtttatgccggcggcgaccagactgtacatggtcacgcactggataccacgctgaatgggggataccagtatgtgcacaacggcggtacagcgtctgacactgttgtgaacagtgacggctggcagattgtcaaaaacgggggtgtggccgggaataccaccgttaatcagaagggcagactgcaggtggacgccggtggtacagccacgaatgtcaccctgaagcagggcggcgcactggttaccagtacggctgcaaccgttaccggcataaaccgcctgggagcattctctgttgtggagggtaaagctgataatgtcgtactggaaaatggcggacgcctggatgtgctgaccggacacacagccactaatacccgcgtggatgatggcggaacgctggatgtccgcaacggtggcaccgccaccaccgtatccatgggaaatggcggtgtactgctggccgattccggtgccgctgtcagtggtacccggagcgacggaaaggcattcagtatcggaggcggtcaggcggatgccctgatgctggaaaaaggcagttcattcacgctgaacgccggtgatacggccacggataccacggtaaatggcggactgttcaccgccaggggcggcacactggcgggcaccaccacgctgaataacggcgccaaaggttaaacacccaagcagacgccgcaatatcagcaccaacagaaaggttaagactactttctgcctttgcgagaacagcaccagaagatagagcgacaggcaagtagcaat

SEQ ID NO: 6 - DNA, 1863 bp, Artificial Sequence
  Synthetic reporter polynucleotide
  misc_feature (1)..(1): 5' Biotinylation
attgcuacttgcctgtcgctctatcttctggtgctgttcagggaacaaaccaagttacgtttaacctacttgcctgtcgctctatcttcggcgtctgcttgggtgtttaaccgtctctcttgtccgtgcaatagctcaataatagaataaaacgatcaatatctattttatcgatcgtttatatcgatcgataagctaataataacctttgtcagtaacatgcacagatacgtacagaaagacattcagggaacaacagaaccacaattcagaaactcccacagccggacctccggcactgtaaccctttacctgccggtatccacgtttgtgggtaccggcttttttattcaccctcaatctaaggaaaagctgatgaaacgacatctgaatacctgctacaggctggtatggaatcacatgacgggcgctttcgtggttgcctccgaactggcccgcgcacggggtaaacgtggcggtgtggcggttgcactgtctcttgccgcagtcacgtcactcccggtgctggctgctgacatcgttgtgcacccgggagaaaccgtgaacggcggaacactggcaaatcatgacaaccagattgtcttcggtacgaccaacggaatgaccatcagtaccgggctggagtatgggccggataacgaggccaataccggcgggcaatgggtacaggatggcggaacagccaacaaaacgactgtcaccagtggtggtcttcagagagtgaaccccggtggaagtgtctcagacacggttatcagtgccggaggcggacagagccttcagggacgggctgtgaacaccacgctgaatggtggcgaacagtggatgcatgagggggcgatagccacaggaaccgtcattaatgataagggctggcaggtcgtcaagcccggtacagtggcaacggataccgttgttaataccggggcggaagggggaccggatgcagaaaacggtgataccgggcagtttgttcgcggggatgccgtacgcacaaccatcaataaaaacggtcgccagattgtgagagctgaaggaacggcaaataccactgtggtttatgccggcggcgaccagactgtacatggtcacgcactggataccacgctgaatgggggataccagtatgtgcacaacggcggtacagcgtctgacactgttgtgaacagtgacggctggcagattgtcaaaaacgggggtgtggccgggaataccaccgttaatcagaagggcagactgcaggtggacgccggtggtacagccacgaatgtcaccctgaagcagggcggcgcactggttaccagtacggctgcaaccgttaccggcataaaccgcctgggagcattctctgttgtggagggtaaagctgataatgtcgtactggaaaatggcggacgcctggatgtgctgaccggacacacagccactaatacccgcgtggatgatggcggaacgctggatgtccgcaacggtggcaccgccaccaccgtatccatgggaaatggcggtgtactgctggccgattccggtgccgctgtcagtggtacccggagcgacggaaaggcattcagtatcggaggcggtcaggcggatgccctgatgctggaaaaaggcagttcattcacgctgaacgccggtgatacggccacggataccacggtaaatggcggactgttcaccgccaggggcggcacactggcgggcaccaccacgctgaataacggcgccaaaggttaaacacccaagcagacgccgcaatatcagcaccaacagaaaggttaaacgtaacttggtttgttccctgaacagcaccagaagatagagcgacaggcaagtagcaat

SEQ ID NO: 7 - DNA, 1863 bp, Artificial Sequence
  Synthetic reporter polynucleotide
  misc_feature (1)..(1): 5' Biotinylation
attgcuacttgcctgtcgctctatcttctggtgctggttcctcgtgcagtgtcaagagatttaacctacttgcctgtcgctctatcttcggcgtctgcttgggtgtttaaccgtctctcttgtccgtgcaatagctcaataatagaataaaacgatcaatatctattttatcgatcgtttatatcgatcgataagctaataataacctttgtcagtaacatgcacagatacgtacagaaagacattcagggaacaacagaaccacaattcagaaactcccacagccggacctccggcactgtaaccctttacctgccggtatccacgtttgtgggtaccggcttttttattcaccctcaatctaaggaaaagctgatgaaacgacatctgaatacctgctacaggctggtatggaatcacatgacgggcgctttcgtggttgcctccgaactggcccgcgcacggggtaaacgtggcggtgtggcggttgcactgtctcttgccgcagtcacgtcactcccggtgctggctgctgacatcgttgtgcacccgggagaaaccgtgaacggcggaacactggcaaatcatgacaaccagattgtcttcggtacgaccaacggaatgaccatcagtaccgggctggagtatgggccggataacgaggccaataccggcgggcaatgggtacaggatggcggaacagccaacaaaacgactgtcaccagtggtggtcttcagagagtgaaccccggtggaagtgtctcagacacggttatcagtgccggaggcggacagagccttcagggacgggctgtgaacaccacgctgaatggtggcgaacagtggatgcatgagggggcgatagccacaggaaccgtcattaatgataagggctggcaggtcgtcaagcccggtacagtggcaacggataccgttgttaataccggggcggaagggggaccggatgcagaaaacggtgataccgggcagtttgttcgcggggatgccgtacgcacaaccatcaataaaaacggtcgccagattgtgagagctgaaggaacggcaaataccactgtggtttatgccggcggcgaccagactgtacatggtcacgcactggataccacgctgaatgggggataccagtatgtgcacaacggcggtacagcgtctgacactgttgtgaacagtgacggctggcagattgtcaaaaacgggggtgtggccgggaataccaccgttaatcagaagggcagactgcaggtggacgccggtggtacagccacgaatgtcaccctgaagcagggcggcgcactggttaccagtacggctgcaaccgttaccggcataaaccgcctgggagcattctctgttgtggagggtaaagctgataatgtcgtactggaaaatggcggacgcctggatgtgctgaccggacacacagccactaatacccgcgtggatgatggcggaacgctggatgtccgcaacggtggcaccgccaccaccgtatccatgggaaatggcggtgtactgctggccgattccggtgccgctgtcagtggtacccggagcgacggaaaggcattcagtatcggaggcggtcaggcggatgccctgatgctggaaaaaggcagttcattcacgctgaacgccggtgatacggccacggataccacggtaaatggcggactgttcaccgccaggggcggcacactggcgggcaccaccacgctgaataacggcgccaaaggttaaacacccaagcagacgccgcaatatcagcaccaacagaaaggttaaatctcttgacactgcacgaggaaccagcaccagaagatagagcgacaggcaagtagcaat

SEQ ID NO: 8 - DNA, 1863 bp, Artificial Sequence
  Synthetic reporter polynucleotide
  misc_feature (1)..(1): 5' Biotinylation
attgcuacttgcctgtcgctctatcttctggtgctgttgcgtcctgttacgagaactcatttaacctacttgcctgtcgctctatcttcggcgtctgcttgggtgtttaaccgtctctcttgtccgtgcaatagctcaataatagaataaaacgatcaatatctattttatcgatcgtttatatcgatcgataagctaataataacctttgtcagtaacatgcacagatacgtacagaaagacattcagggaacaacagaaccacaattcagaaactcccacagccggacctccggcactgtaaccctttacctgccggtatccacgtttgtgggtaccggcttttttattcaccctcaatctaaggaaaagctgatgaaacgacatctgaatacctgctacaggctggtatggaatcacatgacgggcgctttcgtggttgcctccgaactggcccgcgcacggggtaaacgtggcggtgtggcggttgcactgtctcttgccgcagtcacgtcactcccggtgctggctgctgacatcgttgtgcacccgggagaaaccgtgaacggcggaacactggcaaatcatgacaaccagattgtcttcggtacgaccaacggaatgaccatcagtaccgggctggagtatgggccggataacgaggccaataccggcgggcaatgggtacaggatggcggaacagccaacaaaacgactgtcaccagtggtggtcttcagagagtgaaccccggtggaagtgtctcagacacggttatcagtgccggaggcggacagagccttcagggacgggctgtgaacaccacgctgaatggtggcgaacagtggatgcatgagggggcgatagccacaggaaccgtcattaatgataagggctggcaggtcgtcaagcccggtacagtggcaacggataccgttgttaataccggggcggaagggggaccggatgcagaaaacggtgataccgggcagtttgttcgcggggatgccgtacgcacaaccatcaataaaaacggtcgccagattgtgagagctgaaggaacggcaaataccactgtggtttatgccggcggcgaccagactgtacatggtcacgcactggataccacgctgaatgggggataccagtatgtgcacaacggcggtacagcgtctgacactgttgtgaacagtgacggctggcagattgtcaaaaacgggggtgtggccgggaataccaccgttaatcagaagggcagactgcaggtggacgccggtggtacagccacgaatgtcaccctgaagcagggcggcgcactggttaccagtacggctgcaaccgttaccggcataaaccgcctgggagcattctctgttgtggagggtaaagctgataatgtcgtactggaaaatggcggacgcctggatgtgctgaccggacacacagccactaatacccgcgtggatgatggcggaacgctggatgtccgcaacggtggcaccgccaccaccgtatccatgggaaatggcggtgtactgctggccgattccggtgccgctgtcagtggtacccggagcgacggaaaggcattcagtatcggaggcggtcaggcggatgccctgatgctggaaaaaggcagttcattcacgctgaacgccggtgatacggccacggataccacggtaaatggcggactgttcaccgccaggggcggcacactggcgggcaccaccacgctgaataacggcgccaaaggttaaacacccaagcagacgccgcaatatcagcaccaacagaaaggttaaatgagttctcgtaacaggacgcaacagcaccagaagatagagcgacaggcaagtagcaat

SEQ ID NO: 9 - DNA, 1863 bp, Artificial Sequence; identical to SEQ ID NO: 1
  Synthetic reporter polynucleotide
  misc_feature (1)..(1): 5' Biotinylation

SEQ ID NO: 10 - DNA, 1863 bp, Artificial Sequence; identical to SEQ ID NO: 2
  Synthetic reporter polynucleotide
  misc_feature (1)..(1): 5' Biotinylation

SEQ ID NO: 11 - DNA, 1863 bp, Artificial Sequence; identical to SEQ ID NO: 3
  Synthetic reporter polynucleotide
  misc_feature (1)..(1): 5' Biotinylation

SEQ ID NO: 12 - DNA, 1863 bp, Artificial Sequence
  Synthetic reporter polynucleotide
  misc_feature (1)..(1): 5' Biotinylation
attgcuacttgcctgtcgctctatcttctggtgctgttcggattctatcgtgtttccctattaacctacttgcctgtcgctctatcttcggcgtctgcttgggtgtttaaccgtctctcttgtccgtgcaatagctcaataatagaataaaacgatcaatatctattttatcgatcgtttatatcgatcgataagctaataataacctttgtcagtaacatgcacagatacgtacagaaagacattcagggaacaacagaaccacaattcagaaactcccacagccggacctccggcactgtaaccctttacctgccggtatccacgtttgtgggtaccggcttttttattcaccctcaatctaaggaaaagctgatgaaacgacatctgaatacctgctacaggctggtatggaatcacatgacgggcgctttcgtggttgcctccgaactggcccgcgcacggggtaaacgtggcggtgtggcggttgcactgtctcttgccgcagtcacgtcactcccggtgctggctgctgacatcgttgtgcacccgggagaaaccgtgaacggcggaacactggcaaatcatgacaaccagattgtcttcggtacgaccaacggaatgaccatcagtaccgggctggagtatgggccggataacgaggccaataccggcgggcaatgggtacaggatggcggaacagccaacaaaacgactgtcaccagtggtggtcttcagagagtgaaccccggtggaagtgtctcagacacggttatcagtgccggaggcggacagagccttcagggacgggctgtgaacaccacgctgaatggtggcgaacagtggatgcatgagggggcgatagccacaggaaccgtcattaatgataagggctggcaggtcgtcaagcccggtacagtggcaacggataccgttgttaataccggggcggaagggggaccggatgcagaaaacggtgataccgggcagtttgttcgcggggatgccgtacgcacaaccatcaataaaaacggtcgccagattgtgagagctgaaggaacggcaaataccactgtggtttatgccggcggcgaccagactgtacatggtcacgcactggataccacgctgaatgggggataccagtatgtgcacaacggcggtacagcgtctgacactgttgtgaacagtgacggctggcagattgtcaaaaacgggggtgtggccgggaataccaccgttaatcagaagggcagactgcaggtggacgccggtggtacagccacgaatgtcaccctgaagcagggcggcgcactggttaccagtacggctgcaaccgttaccggcataaaccgcctgggagcattctctgttgtggagggtaaagctgataatgtcgtactggaaaatggcggacgcctggatgtgctgaccggacacacagccactaatacccgcgtggatgatggcggaacgctggatgtccgcaacggtggcaccgccaccaccgtatccatgggaaatggcggtgtactgctggccgattccggtgccgctgtcagtggtacccggagcgacggaaaggcattcagtatcggaggcggtcaggcggatgccctgatgctggaaaaaggcagttcattcacgctgaacgccggtgatacggccacggataccacggtaaatggcggactgttcaccgccaggggcggcacactggcgggcaccaccacgctgaataacggcgccaaaggttaaacacccaagcagacgccgcaatatcagcaccaacagaaaggttaatagggaaacacgatagaatccgaacagcaccagaagatagagcgacaggcaagtagcaat

SEQ ID NO: 13 - DNA, 1863 bp, Artificial Sequence; identical to SEQ ID NO: 4
  Synthetic reporter polynucleotide
  misc_feature (1)..(1): 5' Biotinylation

SEQ ID NO: 14 - DNA, 1863 bp, Artificial Sequence; identical to SEQ ID NO: 5
  Synthetic reporter polynucleotide
  misc_feature (1)..(1): 5' Biotinylation

SEQ ID NO: 15 - DNA, 1863 bp, Artificial Sequence; identical to SEQ ID NO: 6
  Synthetic reporter polynucleotide
  misc_feature (1)..(1): 5' Biotinylation

SEQ ID NO: 16 - DNA, 1863 bp, Artificial Sequence
  Synthetic reporter polynucleotide
  misc_feature (1)..(1): 5' Biotinylation
attgcuacttgcctgtcgctctatcttctggtgctgaagcgttgaaacctttgtcctctcttaacctacttgcctgtcgctctatcttcggcgtctgcttgggtgtttaaccgtctctcttgtccgtgcaatagctcaataatagaataaaacgatcaatatctattttatcgatcgtttatatcgatcgataagctaataataacctttgtcagtaacatgcacagatacgtacagaaagacattcagggaacaacagaaccacaattcagaaactcccacagccggacctccggcactgtaaccctttacctgccggtatccacgtttgtgggtaccggcttttttattcaccctcaatctaaggaaaagctgatgaaacgacatctgaatacctgctacaggctggtatggaatcacatgacgggcgctttcgtggttgcctccgaactggcccgcgcacggggtaaacgtggcggtgtggcggttgcactgtctcttgccgcagtcacgtcactcccggtgctggctgctgacatcgttgtgcacccgggagaaaccgtgaacggcggaacactggcaaatcatgacaaccagattgtcttcggtacgaccaacggaatgaccatcagtaccgggctggagtatgggccggataacgaggccaataccggcgggcaatgggtacaggatggcggaacagccaacaaaacgactgtcaccagtggtggtcttcagagagtgaaccccggtggaagtgtctcagacacggttatcagtgccggaggcggacagagccttcagggacgggctgtgaacaccacgctgaatggtggcgaacagtggatgcatgagggggcgatagccacaggaaccgtcattaatgataagggctggcaggtcgtcaagcccggtacagtggcaacggataccgttgttaataccggggcggaagggggaccggatgcagaaaacggtgataccgggcagtttgttcgcggggatgccgtacgcacaaccatcaataaaaacggtcgccagattgtgagagctgaaggaacggcaaataccactgtggtttatgccggcggcgaccagactgtacatggtcacgcactggataccacgctgaatgggggataccagtatgtgcacaacggcggtacagcgtctgacactgttgtgaacagtgacggctggcagattgtcaaaaacgggggtgtggccgggaataccaccgttaatcagaagggcagactgcaggtggacgccggtggtacagccacgaatgtcaccctgaagcagggcggcgcactggttaccagtacggctgcaaccgttaccggcataaaccgcctgggagcattctctgttgtggagggtaaagctgataatgtcgtactggaaaatggcggacgcctggatgtgctgaccggacacacagccactaatacccgcgtggatgatggcggaacgctggatgtccgcaacggtggcaccgccaccaccgtatccatgggaaatggcggtgtactgctggccgattccggtgccgctgtcagtggtacccggagcgacggaaaggcattcagtatcggaggcggtcaggcggatgccctgatgctggaaaaaggcagttcattcacgctgaacgccggtgatacggccacggataccacggtaaatggcggactgttcaccgccaggggcggcacactggcgggcaccaccacgctgaataacggcgccaaaggttaaacacccaagcagacgccgcaatatcagcaccaacagaaaggttaagagaggacaaaggtttcaacgcttcagcaccagaagatagagcgacaggcaagtagcaat

SEQ ID NO: 17 - DNA, 1863 bp, Artificial Sequence; identical to SEQ ID NO: 16
  Synthetic reporter polynucleotide
  misc_feature (1)..(1): 5' Biotinylation

SEQ ID NO: 18 - DNA, 1863 bp, Artificial Sequence
  Synthetic reporter polynucleotide
  misc_feature (1)..(1): 5' Biotinylation
attgcuacttgcctgtcgctctatcttctggtgctgcaggtagaaagaagcagaatcggattaacctacttgcctgtcgctctatcttcggcgtctgcttgggtgtttaaccgtctctcttgtccgtgcaatagctcaataatagaataaaacgatcaatatctattttatcgatcgtttatatcgatcgataagctaataataacctttgtcagtaacatgcacagatacgtacagaaagacattcagggaacaacagaaccacaattcagaaactcccacagccggacctccggcactgtaaccctttacctgccggtatccacgtttgtgggtaccggcttttttattcaccctcaatctaaggaaaagctgatgaaacgacatctgaatacctgctacaggctggtatggaatcacatgacgggcgctttcgtggttgcctccgaactggcccgcgcacggggtaaacgtggcggtgtggcggttgcactgtctcttgccgcagtcacgtcactcccggtgctggctgctgacatcgttgtgcacccgggagaaaccgtgaacggcggaacactggcaaatcatgacaaccagattgtcttcggtacgaccaacggaatgaccatcagtaccgggctggagtatgggccggataacgaggccaataccggcgggcaatgggtacaggatggcggaacagccaacaaaacgactgtcaccagtggtggtcttcagagagtgaaccccggtggaagtgtctcagacacggttatcagtgccggaggcggacagagccttcagggacgggctgtgaacaccacgctgaatggtggcgaacagtggatgcatgagggggcgatagccacaggaaccgtcattaatgataagggctggcaggtcgtcaagcccggtacagtggcaacggataccgttgttaataccggggcggaagggggaccggatgcagaaaacggtgataccgggcagtttgttcgcggggatgccgtacgcacaaccatcaataaaaacggtcgccagattgtgagagctgaaggaacggcaaataccactgtggtttatgccggcggcgaccagactgtacatggtcacgcactggataccacgctgaatgggggataccagtatgtgcacaacggcggtacagcgtctgacactgttgtgaacagtgacggctggcagattgtcaaaaacgggggtgtggccgggaataccaccgttaatcagaagggcagactgcaggtggacgccggtggtacagccacgaatgtcaccctgaagcagggcggcgcactggttaccagtacggctgcaaccgttaccggcataaaccgcctgggagcattctctgttgtggagggtaaagctgataatgtcgtactggaaaatggcggacgcctggatgtgctgaccggacacacagccactaatacccgcgtggatgatggcggaacgctggatgtccgcaacggtggcaccgccaccaccgtatccatgggaaatggcggtgtactgctggccgattccggtgccgctgtcagtggtacccggagcgacggaaaggcattcagtatcggaggcggtcaggcggatgccctgatgctggaaaaaggcagttcattcacgctgaacgccggtgatacggccacggataccacggtaaatggcggactgttcaccgccaggggcggcacactggcgggcaccaccacgctgaataacggcgccaaaggttaaacacccaagcagacgccgcaatatcagcaccaacagaaaggttaatccgattctgcttctttctacctgcagcaccagaagatagagcgacaggcaagtagcaat

SEQ ID NO: 19 - DNA, 1863 bp, Artificial Sequence
  Synthetic reporter polynucleotide
  misc_feature (1)..(1): 5' Biotinylation
attgcuacttgcctgtcgctctatcttctggtgctgagaacgacttccatactcgtgtgattaacctacttgcctgtcgctctatcttcggcgtctgcttgggtgtttaaccgtctctcttgtccgtgcaatagctcaataatagaataaaacgatcaatatctattttatcgatcgtttatatcgatcgataagctaataataacctttgtcagtaacatgcacagatacgtacagaaagacattcagggaacaacagaaccacaattcagaaactcccacagccggacctccggcactgtaaccctttacctgccggtatccacgtttgtgggtaccggcttttttattcaccctcaatctaaggaaaagctgatgaaacgacatctgaatacctgctacaggctggtatggaatcacatgacgggcgctttcgtggttgcctccgaactggcccgcgcacggggtaaacgtggcggtgtggcggttgcactgtctcttgccgcagtcacgtcactcccggtgctggctgctgacatcgttgtgcacccgggagaaaccgtgaacggcggaacactggcaaatcatgacaaccagattgtcttcggtacgaccaacggaatgaccatcagtaccgggctggagtatgggccggataacgaggccaataccggcgggcaatgggtacaggatggcggaacagccaacaaaacgactgtcaccagtggtggtcttcagagagtgaaccccggtggaagtgtctcagacacggttatcagtgccggaggcggacagagccttcagggacgggctgtgaacaccacgctgaatggtggcgaacagtggatgcatgagggggcgatagccacaggaaccgtcattaatgataagggctggcaggtcgtcaagcccggtacagtggcaacggataccgttgttaataccggggcggaagggggaccggatgcagaaaacggtgataccgggcagtttgttcgcggggatgccgtacgcacaaccatcaataaaaacggtcgccagattgtgagagctgaaggaacggcaaataccactgtggtttatgccggcggcgaccagactgtacatggtcacgcactggataccacgctgaatgggggataccagtatgtgcacaacggcggtacagcgtctgacactgttgtgaacagtgacggctggcagattgtcaaaaacgggggtgtggccgggaataccaccgttaatcagaagggcagactgcaggtggacgccggtggtacagccacgaatgtcaccctgaagcagggcggcgcactggttaccagtacggctgcaaccgttaccggcataaaccgcctgggagcattctctgttgtggagggtaaagctgataatgtcgtactggaaaatggcggacgcctggatgtgctgaccggacacacagccactaatacccgcgtggatgatggcggaacgctggatgtccgcaacggtggcaccgccaccaccgtatccatgggaaatggcggtgtactgctggccgattccggtgccgctgtcagtggtacccggagcgacggaaaggcattcagtatcggaggcggtcaggcggatgccctgatgctggaaaaaggcagttcattcacgctgaacgccggtgatacggccacggataccacggtaaatggcggactgttcaccgccaggggcggcacactggcgggcaccaccacgctgaataacggcgccaaaggttaaacacccaagcagacgccgcaatatcagcaccaacagaaaggttaatcacacgagtatggaagtcgttctcagcaccagaagatagagcgacaggcaagtagcaat

SEQ ID NO: 20 - DNA, 1863 bp, Artificial Sequence
  Synthetic reporter polynucleotide
  misc_feature (1)..(1): 5' Biotinylation
attgcuacttgcctgtcgctctatcttctggtgctgaggtctacctcgctaacaccactgttaacctacttgcctgtcgctctatcttcggcgtctgcttgggtgtttaaccgtctctcttgtccgtgcaatagctcaataatagaataaaacgatcaatatctattttatcgatcgtttatatcgatcgataagctaataataacctttgtcagtaacatgcacagatacgtacagaaagacattcagggaacaacagaaccacaattcagaaactcccacagccggacctccggcactgtaaccctttacctgccggtatccacgtttgtgggtaccggcttttttattcaccctcaatctaaggaaaagctgatgaaacgacatctgaatacctgctacaggctggtatggaatcacatgacgggcgctttcgtggttgcctccgaactggcccgcgcacggggtaaacgtggcggtgtggcggttgcactgtctcttgccgcagtcacgtcactcccggtgctggctgctgacatcgttgtgcacccgggagaaaccgtgaacggcggaacactggcaaatcatgacaaccagattgtcttcggtacgaccaacggaatgaccatcagtaccgggctggagtatgggccggataacgaggccaataccggcgggcaatgggtacaggatggcggaacagccaacaaaacgactgtcaccagtggtggtcttcagagagtgaaccccggtggaagtgtctcagacacggttatcagtgccggaggcggacagagccttcagggacgggctgtgaacaccacgctgaatggtggcgaacagtggatgcatgagggggcgatagccacaggaaccgtcattaatgataagggctggcaggtcgtcaagcccggtacagtggcaacggataccgttgttaataccggggcggaagggggaccggatgcagaaaacggtgataccgggcagtttgttcgcggggatgccgtacgcacaaccatcaataaaaacggtcgccagattgtgagagctgaaggaacggcaaataccactgtggtttatgccggcggcgaccagactgtacatggtcacgcactggataccacgctgaatgggggataccagtatgtgcacaacggcggtacagcgtctgacactgttgtgaacagtgacggctggcagattgtcaaaaacgggggtgtggccgggaataccaccgttaatcagaagggcagactgcaggtggacgccggtggtacagccacgaatgtcaccctgaagcagggcggcgcactggttaccagtacggctgcaaccgttaccggcataaaccgcctgggagcattctctgttgtggagggtaaagctgataatgtcgtactggaaaatggcggacgcctggatgtgctgaccggacacacagccactaatacccgcgtggatgatggcggaacgctggatgtccgcaacggtggcaccgccaccaccgtatccatgggaaatggcggtgtactgctggccgattccggtgccgctgtcagtggtacccggagcgacggaaaggcattcagtatcggaggcggtcaggcggatgccctgatgctggaaaaaggcagttcattcacgctgaacgccggtgatacggccacggataccacggtaaatggcggactgttcaccgccaggggcggcacactggcgggcaccaccacgctgaataacggcgccaaaggttaaacacccaagcagacgccgcaatatcagcaccaacagaaaggttaacagtggtgttagcgaggtagacctcagcaccagaagatagagcgacaggcaagtagcaat

SEQ ID NO: 21 - DNA, 1863 bp, Artificial Sequence
  Synthetic reporter polynucleotide
  misc_feature (1)..(1): 5' Biotinylation
attgcuacttgcctgtcgctctatcttctggtgctgaccctccaggaaagtacctctgatttaacctacttgcctgtcgctctatcttcggcgtctgcttgggtgtttaaccgtctctcttgtccgtgcaatagctcaataatagaataaaacgatcaatatctattttatcgatcgtttatatcgatcgataagctaataataacctttgtcagtaacatgcacagatacgtacagaaagacattcagggaacaacagaaccacaattcagaaactcccacagccggacctccggcactgtaaccctttacctgccggtatccacgtttgtgggtaccggcttttttattcaccctcaatctaaggaaaagctgatgaaacgacatctgaatacctgctacaggctggtatggaatcacatgacgggcgctttcgtggttgcctccgaactggcccgcgcacggggtaaacgtggcggtgtggcggttgcactgtctcttgccgcagtcacgtcactcccggtgctggctgctgacatcgttgtgcacccgggagaaaccgtgaacggcggaacactggcaaatcatgacaaccagattgtcttcggtacgaccaacggaatgaccatcagtaccgggctggagtatgggccggataacgaggccaataccggcgggcaatgggtacaggatggcggaacagccaacaaaacgactgtcaccagtggtggtcttcagagagtgaaccccggtggaagtgtctcagacacggttatcagtgccggaggcggacagagccttcagggacgggctgtgaacaccacgctgaatggtggcgaacagtggatgcatgagggggcgatagccacaggaaccgtcattaatgataagggctggcaggtcgtcaagcccggtacagtggcaacggataccgttgttaataccggggcggaagggggaccggatgcagaaaacggtgataccgggcagtttgttcgcggggatgccgtacgcacaaccatcaataaaaacggtcgccagattgtgagagctgaaggaacggcaaataccactgtggtttatgccggcggcgaccagactgtacatggtcacgcactggataccacgctgaatgggggataccagtatgtgcacaacggcggtacagcgtctgacactgttgtgaacagtgacggctggcagattgtcaaaaacgggggtgtggccgggaataccaccgttaatcagaagggcagactgcaggtggacgccggtggtacagccacgaatgtcaccctgaagcagggcggcgcactggttaccagtacggctgcaaccgttaccggcataaaccgcctgggagcattctctgttgtggagggtaaagctgataatgtcgtactggaaaatggcggacgcctggatgtgctgaccggacacacagccactaatacccgcgtggatgatggcggaacgctggatgtccgcaacggtggcaccgccaccaccgtatccatgggaaatggcggtgtactgctggccgattccggtgccgctgtcagtggtacccggagcgacggaaaggcattcagtatcggaggcggtcaggcggatgccctgatgctggaaaaaggcagttcattcacgctgaacgccggtgatacggccacggataccacggtaaatggcggactgttcaccgccaggggcggcacactggcgggcaccaccacgctgaataacggcgccaaaggttaaacacccaagcagacgccgcaatatcagcaccaacagaaaggttaaatcagaggtactttcctggagggtcagcaccagaagatagagcgacaggcaagtagcaat

SEQ ID NO: 22 - DNA, 1863 bp, Artificial Sequence; identical to SEQ ID NO: 7
  Synthetic reporter polynucleotide
  misc_feature (1)..(1): 5' Biotinylation

SEQ ID NO: 23 - DNA, 1863 bp, Artificial Sequence; identical to SEQ ID NO: 8
  Synthetic reporter polynucleotide
  misc_feature (1)..(1): 5' Biotinylation

SEQ ID NO: 24 - DNA, 1863 bp, Artificial Sequence
  Synthetic reporter polynucleotide
  misc_feature (1)..(1): 5' Biotinylation
attgcuacttgcctgtcgctctatcttctggtgctgcttactacccagtgaacctcctcgttaacctacttgcctgtcgctctatcttcggcgtctgcttgggtgtttaaccgtctctcttgtccgtgcaatagctcaataatagaataaaacgatcaatatctattttatcgatcgtttatatcgatcgataagctaataataacctttgtcagtaacatgcacagatacgtacagaaagacattcagggaacaacagaaccacaattcagaaactcccacagccggacctccggcactgtaaccctttacctgccggtatccacgtttgtgggtaccggcttttttattcaccctcaatctaaggaaaagctgatgaaacgacatctgaatacctgctacaggctggtatggaatcacatgacgggcgctttcgtggttgcctccgaactggcccgcgcacggggtaaacgtggcggtgtggcggttgcactgtctcttgccgcagtcacgtcactcccggtgctggctgctgacatcgttgtgcacccgggagaaaccgtgaacggcggaacactggcaaatcatgacaaccagattgtcttcggtacgaccaacggaatgaccatcagtaccgggctggagtatgggccggataacgaggccaataccggcgggcaatgggtacaggatggcggaacagccaacaaaacgactgtcaccagtggtggtcttcagagagtgaaccccggtggaagtgtctcagacacggttatcagtgccggaggcggacagagccttcagggacgggctgtgaacaccacgctgaatggtggcgaacagtggatgcatgagggggcgatagccacaggaaccgtcattaatgataagggctggcaggtcgtcaagcccggtacagtggcaacggataccgttgttaataccggggcggaagggggaccggatgcagaaaacggtgataccgggcagtttgttcgcggggatgccgtacgcacaaccatcaataaaaacggtcgccagattgtgagagctgaaggaacggcaaataccactgtggtttatgccggcggcgaccagactgtacatggtcacgcactggataccacgctgaatgggggataccagtatgtgcacaacggcggtacagcgtctgacactgttgtgaacagtgacggctggcagattgtcaaaaacgggggtgtggccgggaataccaccgttaatcagaagggcagactgcaggtggacgccggtggtacagccacgaatgtcaccctgaagcagggcggcgcactggttaccagtacggctgcaaccgttaccggcataaaccgcctgggagcattctctgttgtggagggtaaagctgataatgtcgtactggaaaatggcggacgcctggatgtgctgaccggacacacagccactaatacccgcgtggatgatggcggaacgctggatgtccgcaacggtggcaccgccaccaccgtatccatgggaaatggcggtgtactgctggccgattccggtgccgctgtcagtggtacccggagcgacggaaaggcattcagtatcggaggcggtcaggcggatgccctgatgctggaaaaaggcagttcattcacgctgaacgccggtgatacggccacggataccacggtaaatggcggactgttcaccgccaggggcggcacactggcgggcaccaccacgctgaataacggcgccaaaggttaaacacccaagcagacgccgcaatatcagcaccaacagaaaggttaacgaggaggttcactgggtagtaagcagcaccagaagatagagcgacaggcaagtagcaat

SEQ ID NO: 25 - DNA, 1863 bp, Artificial Sequence
  Synthetic reporter polynucleotide
  misc_feature (1)..(1): 5' Biotinylation
attgcuacttgcctgtcgctctatcttctggtgctggcatagttctgcatgatgggttagttaacctacttgcctgtcgctctatcttcggcgtctgcttgggtgtttaaccgtctctcttgtccgtgcaatagctcaataatagaataaaacgatcaatatctattttatcgatcgtttatatcgatcgataagctaataataacctttgtcagtaacatgcacagatacgtacagaaagacattcagggaacaacagaaccacaattcagaaactcccacagccggacctccggcactgtaaccctttacctgccggtatccacgtttgtgggtaccggcttttttattcaccctcaatctaaggaaaagctgatgaaacgacatctgaatacctgctacaggctggtatggaatcacatgacgggcgctttcgtggttgcctccgaactggcccgcgcacggggtaaacgtggcggtgtggcggttgcactgtctcttgccgcagtcacgtcactcccggtgctggctgctgacatcgttgtgcacccgggagaaaccgtgaacggcggaacactggcaaatcatgacaaccagattgtcttcggtacgaccaacggaatgaccatcagtaccgggctggagtatgggccggataacgaggccaataccggcgggcaatgggtacaggatggcggaacagccaacaaaacgactgtcaccagtggtggtcttcagagagtgaaccccggtggaagtgtctcagacacggttatcagtgccggaggcggacagagccttcagggacgggctgtgaacaccacgctgaatggtggcgaacagtggatgcatgagggggcgatagccacaggaaccgtcattaatgataagggctggcaggtcgtcaagcccggtacagtggcaacggataccgttgttaataccggggcggaagggggaccggatgcagaaaacggtgataccgggcagtttgttcgcggggatgccgtacgcacaaccatcaataaaaacggtcgccagattgtgagagctgaaggaacggcaaataccactgtggtttatgccggcggcgaccagactgtacatggtcacgcactggataccacgctgaatgggggataccagtatgtgcacaacggcggtacagcgtctgacactgttgtgaacagtgacggctggcagattgtcaaaaacgggggtgtggccgggaataccaccgttaatcagaagggcagactgcaggtggacgccggtggtacagccacgaatgtcaccctgaagcagggcggcgcactggttaccagtacggctgcaaccgttaccggcataaaccgcctgggagcattctctgttgtggagggtaaagctgataatgtcgtactggaaaatggcggacgcctggatgtgctgaccggacacacagccactaatacccgcgtggatgatggcggaacgctggatgtccgcaacggtggcaccgccaccaccgtatccatgggaaatggcggtgtactgctggccgattccggtgccgctgtcagtggtacccggagcgacggaaaggcattcagtatcggaggcggtcaggcggatgccctgatgctggaaaaaggcagttcattcacgctgaacgccggtgatacggccacggataccacggtaaatggcggactgttcaccgccaggggcggcacactggcgggcaccaccacgctgaataacggcgccaaaggttaaacacccaagcagacgccgcaatatcagcaccaacagaaaggttaactaacccatcatgcagaactatgccagcaccagaagatagagcgacaggcaagtagcaat

SEQ ID NO: 26 - DNA, 1863 bp, Artificial Sequence
  Synthetic reporter polynucleotide
  misc_feature (1)..(1): 5' Biotinylation
attgcuacttgcctgtcgctctatcttctggtgctgcatacagcgactacgcattctcatttaacctacttgcctgtcgctctatcttcggcgtctgcttgggtgtttaaccgtctctcttgtccgtgcaatagctcaataatagaataaaacgatcaatatctattttatcgatcgtttatatcgatcgataagctaataataacctttgtcagtaacatgcacagatacgtacagaaagacattcagggaacaacagaaccacaattcagaaactcccacagccggacctccggcactgtaaccctttacctgccggtatccacgtttgtgggtaccggcttttttattcaccctcaatctaaggaaaagctgatgaaacgacatctgaatacctgctacaggctggtatggaatcacatgacgggcgctttcgtggttgcctccgaactggcccgcgcacggggtaaacgtggcggtgtggcggttgcactgtctcttgccgcagtcacgtcactcccggtgctggctgctgacatcgttgtgcacccgggagaaaccgtgaacggcggaacactggcaaatcatgacaaccagattgtcttcggtacgaccaacggaatgaccatcagtaccgggctggagtatgggccggataacgaggccaataccggcgggcaatgggtacaggatggcggaacagccaacaaaacgactgtcaccagtggtggtcttcagagagtgaaccccggtggaagtgtctcagacacggttatcagtgccggaggcggacagagccttcagggacgggctgtgaacaccacgctgaatggtggcgaacagtggatgcatgagggggcgatagccacaggaaccgtcattaatgataagggctggcaggtcgtcaagcccggtacagtggcaacggataccgttgttaataccggggcggaagggggaccggatgcagaaaacggtgataccgggcagtttgttcgcggggatgccgtacgcacaaccatcaataaaaacggtcgccagattgtgagagctgaaggaacggcaaataccactgtggtttatgccggcggcgaccagactgtacatggtcacgcactggataccacgctgaatgggggataccagtatgtgcacaacggcggtacagcgtctgacactgttgtgaacagtgacggctggcagattgtcaaaaacgggggtgtggccgggaataccaccgttaatcagaagggcagactgcaggtggacgccggtggtacagccacgaatgtcaccctgaagcagggcggcgcactggttaccagtacggctgcaaccgttaccggcataaaccgcctgggagcattctctgttgtggagggtaaagctgataatgtcgtactggaaaatggcggacgcctggatgtgctgaccggacacacagccactaatacccgcgtggatgatggcggaacgctggatgtccgcaacggtggcaccgccaccaccgtatccatgggaaatggcggtgtactgctggccgattccggtgccgctgtcagtggtacccggagcgacggaaaggcattcagtatcggaggcggtcaggcggatgccctgatgctggaaaaaggcagttcattcacgctgaacgccggtgatacggccacggataccacggtaaatggcggactgttcaccgccaggggcggcacactggcgggcaccaccacgctgaataacggcgccaaaggttaaacacccaagcagacgccgcaatatcagcaccaacagaaaggttaaatgagaatgcgtagtcgctgtatgcagcaccagaagatagagcgacaggcaagtagcaat

SEQ ID NO: 27 - DNA, 1863 bp, Artificial Sequence
  Synthetic reporter polynucleotide
  misc_feature (1)..(1): 5' Biotinylation
attgcuacttgcctgtcgctctatcttctggtgctgcgacggttagattcacctcttacattaacctacttgcctgtcgctctatcttcggcgtctgcttgggtgtttaaccgtctctcttgtccgtgcaatagctcaataatagaataaaacgatcaatatctattttatcgatcgtttatatcgatcgataagctaataataacctttgtcagtaacatgcacagatacgtacagaaagacattcagggaacaacagaaccacaattcagaaactcccacagccggacctccggcactgtaaccctttacctgccggtatccacgtttgtgggtaccggcttttttattcaccctcaatctaaggaaaagctgatgaaacgacatctgaatacctgctacaggctggtatggaatcacatgacgggcgctttcgtggttgcctccgaactggcccgcgcacggggtaaacgtggcggtgtggcggttgcactgtctcttgccgcagtcacgtcactcccggtgctggctgctgacatcgttgtgcacccgggagaaaccgtgaacggcggaacactggcaaatcatgacaaccagattgtcttcggtacgaccaacggaatgaccatcagtaccgggctggagtatgggccggataacgaggccaataccggcgggcaatgggtacaggatggcggaacagccaacaaaacgactgtcaccagtggtggtcttcagagagtgaaccccggtggaagtgtctcagacacggttatcagtgccggaggcggacagagccttcagggacgggctgtgaacaccacgctgaatggtggcgaacagtggatgcatgagggggcgatagccacaggaaccgtcattaatgataagggctggcaggtcgtcaagcccggtacagtggcaacggataccgttgttaataccggggcggaagggggaccggatgcagaaaacggtgataccgggcagtttgttcgcggggatgccgtacgcacaaccatcaataaaaacggtcgccagattgtgagagctgaaggaacggcaaataccactgtggtttatgccggcggcgaccagactgtacatggtcacgcactggataccacgctgaatgggggataccagtatgtgcacaacggcggtacagcgtctgacactgttgtgaacagtgacggctggcagattgtcaaaaacgggggtgtggccgggaataccaccgttaatcagaagggcagactgcaggtggacgccggtggtacagccacgaatgtcaccctgaagcagggcggcgcactggttaccagtacggctgcaaccgttaccggcataaaccgcctgggagcattctctgttgtggagggtaaagctgataatgtcgtactggaaaatggcggacgcctggatgtgctgaccggacacacagccactaatacccgcgtggatgatggcggaacgctggatgtccgcaacggtggcaccgccaccaccgtatccatgggaaatggcggtgtactgctggccgattccggtgccgctgtcagtggtacccggagcgacggaaaggcattcagtatcggaggcggtcaggcggatgccctgatgctggaaaaaggcagttcattcacgctgaacgccggtgatacggccacggataccacggtaaatggcggactgttcaccgccaggggcggcacactggcgggcaccaccacgctgaataacggcgccaaaggttaaacacccaagcagacgccgcaatatcagcaccaacagaaaggttaatgtaagaggtgaatctaaccgtcgcagcaccagaagatagagcgacaggcaagtagcaat

SEQ ID NO: 28 - DNA, 1863 bp, Artificial Sequence
  Synthetic reporter polynucleotide
  misc_feature (1)..(1): 5' Biotinylation
attgcuacttgcctgtcgctctatcttctggtgctgctagacaccttgggttgacagaccttaacctacttgcctgtcgctctatcttcggcgtctgcttgggtgtttaaccgtctctcttgtccgtgcaatagctcaataatagaataaaacgatcaatatctattttatcgatcgtttatatcgatcgataagctaataataacctttgtcagtaacatgcacagatacgtacagaaagacattcagggaacaacagaaccacaattcagaaactcccacagccggacctccggcactgtaaccctttacctgccggtatccacgtttgtgggtaccggcttttttattcaccctcaatctaaggaaaagctgatgaaacgacatctgaatacctgctacaggctggtatggaatcacatgacgggcgctttcgtggttgcctccgaactggcccgcgcacggggtaaacgtggcggtgtggcggttgcactgtctcttgccgcagtcacgtcactcccggtgctggctgctgacatcgttgtgcacccgggagaaaccgtgaacggcggaacactggcaaatcatgacaaccagattgtcttcggtacgaccaacggaatgaccatcagtaccgggctggagtatgggccggataacgaggccaataccggcgggcaatgggtacaggatggcggaacagccaacaaaacgactgtcaccagtggtggtcttcagagagtgaaccccggtggaagtgtctcagacacggttatcagtgccggaggcggacagagccttcagggacgggctgtgaacaccacgctgaatggtggcgaacagtggatgcatgagggggcgatagccacaggaaccgtcattaatgataagggctggcaggtcgtcaagcccggtacagtggcaacggataccgttgttaataccggggcggaagggggaccggatgcagaaaacggtgataccgggcagtttgttcgcggggatgccgtacgcacaaccatcaataaaaacggtcgccagattgtgagagctgaaggaacggcaaataccactgtggtttatgccggcggcgaccagactgtacatggtcacgcactggataccacgctgaatgggggataccagtatgtgcacaacggcggtacagcgtctgacactgttgtgaacagtgacggctggcagattgtcaaaaacgggggtgtggccgggaataccaccgttaatcagaagggcagactgcaggtggacgccggtggtacagccacgaatgtcaccctgaagcagggcggcgcactggttaccagtacggctgcaaccgttaccggcataaaccgcctgggagcattctctgttgtggagggtaaagctgataatgtcgtactggaaaatggcggacgcctggatgtgctgaccggacacacagccactaatacccgcgtggatgatggcggaacgctggatgtccgcaacggtggcaccgccaccaccgtatccatgggaaatggcggtgtactgctggccgattccggtgccgctgtcagtggtacccggagcgacggaaaggcattcagtatcggaggcggtcaggcggatgccctgatgctggaaaaaggcagttcattcacgctgaacgccggtgatacggccacggataccacggtaaatggcggactgttcaccgccaggggcggcacactggcgggcaccaccacgctgaataacggcgccaaaggttaaacacccaagcagacgccgcaatatcagcaccaacagaaaggttaaggtctgtcaacccaaggtgtctagcagcaccagaagatagagcgacaggcaagtagcaat

SEQ ID NO: 29 - DNA, 1863 bp, Artificial Sequence
  Synthetic reporter polynucleotide
  misc_feature (1)..(1): 5' Biotinylation
attgcuacttgcctgtcgctctatcttctggtgctgtcagtgaggatctacttcgacccattaacctacttgcctgtcgctctatcttcggcgtctgcttgggtgtttaaccgtctctcttgtccgtgcaatagctcaataatagaataaaacgatcaatatctattttatcgatcgtttatatcgatcgataagctaataataacctttgtcagtaacatgcacagatacgtacagaaagacattcagggaacaacagaaccacaattcagaaactcccacagccggacctccggcactgtaaccctttacctgccggtatccacgtttgtgggtaccggcttttttattcaccctcaatctaaggaaaagctgatgaaacgacatctgaatacctgctacaggctggtatggaatcacatgacgggcgctttcgtggttgcctccgaactggcccgcgcacggggtaaacgtggcggtgtggcggttgcactgtctcttgccgcagtcacgtcactcccggtgctggctgctgacatcgttgtgcacccgggagaaaccgtgaacggcggaacactggcaaatcatgacaaccagattgtcttcggtacgaccaacggaatgaccatcagtaccgggctggagtatgggccggataacgaggccaataccggcgggcaatgggtacaggatggcggaacagccaacaaaacgactgtcaccagtggtggtcttcagagagtgaaccccggtggaagtgtctcagacacggttatcagtgccggaggcggacagagccttcagggacgggctgtgaacaccacgctgaatggtggcgaacagtggatgcatgagggggcgatagccacaggaaccgtcattaatgataagggctggcaggtcgtcaagcccggtacagtggcaacggataccgttgttaataccggggcggaagggggaccggatgcagaaaacggtgataccgggcagtttgttcgcggggatgccgtacgcacaaccatcaataaaaacggtcgccagattgtgagagctgaaggaacggcaaataccactgtggtttatgccggcggcgaccagactgtacatggtcacgcactggataccacgctgaatgggggataccagtatgtgcacaacggcggtacagcgtctgacactgttgtgaacagtgacggctggcagattgtcaaaaacgggggtgtggccgggaataccaccgttaatcagaagggcagactgcaggtggacgccggtggtacagccacgaatgtcaccctgaagcagggcggcgcactggttaccagtacggctgcaaccgttaccggcataaaccgcctgggagcattctctgttgtggagggtaaagctgataatgtcgtactggaaaatggcggacgcctggatgtgctgaccggacacacagccactaatacccgcgtggatgatggcggaacgctggatgtccgcaacggtggcaccgccaccaccgtatccatgggaaatggcggtgtactgctggccgattccggtgccgctgtcagtggtacccggagcgacggaaaggcattcagtatcggaggcggtcaggcggatgccctgatgctggaaaaaggcagttcattcacgctgaacgccggtgatacggccacggataccacggtaaatggcggactgttcaccgccaggggcggcacactggcgggcaccaccacgctgaataacggcgccaaaggttaaacacccaagcagacgccgcaatatcagcaccaacagaaaggttaatgggtcgaagtagatcctcactgacagcaccagaagatagagcgacaggcaagtagcaat

SEQ ID NO: 30 - DNA, 1863 bp, Artificial Sequence
  Synthetic reporter polynucleotide
  misc_feature (1)..(1): 5' Biotinylation
attgcuacttgcctgtcgctctatcttctggtgctgtgcgtacagcaatcagttacattgttaacctacttgcctgtcgctctatcttcggcgtctgcttgggtgtttaaccgtctctcttgtccgtgcaatagctcaataatagaataaaacgatcaatatctattttatcgatcgtttatatcgatcgataagctaataataacctttgtcagtaacatgcacagatacgtacagaaagacattcagggaacaacagaaccacaattcagaaactcccacagccggacctccggcactgtaaccctttacctgccggtatccacgtttgtgggtaccggcttttttattcaccctcaatctaaggaaaagctgatgaaacgacatctgaatacctgctacaggctggtatggaatcacatgacgggcgctttcgtggttgcctccgaactggcccgcgcacggggtaaacgtggcggtgtggcggttgcactgtctcttgccgcagtcacgtcactcccggtgctggctgctgacatcgttgtgcacccgggagaaaccgtgaacggcggaacactggcaaatcatgacaaccagattgtcttcggtacgaccaacggaatgaccatcagtaccgggctggagtatgggccggataacgaggccaataccggcgggcaatgggtacaggatggcggaacagccaacaaaacgactgtcaccagtggtggtcttcagagagtgaaccccggtggaagtgtctcagacacggttatcagtgccggaggcggacagagccttcagggacgggctgtgaacaccacgctgaatggtggcgaacagtggatgcatgagggggcgatagccacaggaaccgtcattaatgataagggctggcaggtcgtcaagcccggtacagtggcaacggataccgttgttaataccggggcggaagggggaccggatgcagaaaacggtgataccgggcagtttgttcgcggggatgccgtacgcacaaccatcaataaaaacggtcgccagattgtgagagctgaaggaacggcaaataccactgtggtttatgccggcggcgaccagactgtacatggtcacgcactggataccacgctgaatgggggataccagtatgtgcacaacggcggtacagcgtctgacactgttgtgaacagtgacggctggcagattgtcaaaaacgggggtgtggccgggaataccaccgttaatcagaagggcagactgcaggtggacgccggtggtacagccacgaatgtcaccctgaagcagggcggcgcactggttaccagtacggctgcaaccgttaccggcataaaccgcctgggagcattctctgttgtggagggtaaagctgataatgtcgtactggaaaatggcggacgcctggatgtgctgaccggacacacagccactaatacccgcgtggatgatggcggaacgctggatgtccgcaacggtggcaccgccaccaccgtatccatgggaaatggcggtgtactgctggccgattccggtgccgctgtcagtggtacccggagcgacggaaaggcattcagtatcggaggcggtcaggcggatgccctgatgctggaaaaaggcagttcattcacgctgaacgccggtgatacggccacggataccacggtaaatggcggactgttcaccgccaggggcggcacactggcgggcaccaccacgctgaataacggcgccaaaggttaaacacccaagcagacgccgcaatatcagcaccaacagaaaggttaacaatgtaactgattgctgtacgcacagcaccagaagatagagcgacaggcaagtagcaat

SEQ ID NO: 31 - DNA, 1863 bp, Artificial Sequence
  Synthetic reporter polynucleotide
  misc_feature (1)..(1): 5' Biotinylation
attgcuacttgcctgtcgctctatcttctggtgctgccagtagaagtccgacaacgtcatttaacctacttgcctgtcgctctatcttcggcgtctgcttgggtgtttaaccgtctctcttgtccgtgcaatagctcaataatagaataaaacgatcaatatctattttatcgatcgtttatatcgatcgataagctaataataacctttgtcagtaacatgcacagatacgtacagaaagacattcagggaacaacagaaccacaattcagaaactcccacagccggacctccggcactgtaaccctttacctgccggtatccacgtttgtgggtaccggcttttttattcaccctcaatctaaggaaaagctgatgaaacgacatctgaatacctgctacaggctggtatggaatcacatgacgggcgctttcgtggttgcctccgaactggcccgcgcacggggtaaacgtggcggtgtggcggttgcactgtctcttgccgcagtcacgtcactcccggtgctggctgctgacatcgttgtgcacccgggagaaaccgtgaacggcggaacactggcaaatcatgacaaccagattgtcttcggtacgaccaacggaatgaccatcagtaccgggctggagtatgggccggataacgaggccaataccggcgggcaatgggtacaggatggcggaacagccaacaaaacgactgtcaccagtggtggtcttcagagagtgaaccccggtggaagtgtctcagacacggttatcagtgccggaggcggacagagccttcagggacgggctgtgaacaccacgctgaatggtggcgaacagtggatgcatgagggggcgatagccacaggaaccgtcattaatgataagggctggcaggtcgtcaagcccggtacagtggcaacggataccgttgttaataccggggcggaagggggaccggatgcagaaaacggtgataccgggcagtttgttcgcggggatgccgtacgcacaaccatcaataaaaacggtcgccagattgtgagagctgaaggaacggcaaataccactgtggtttatgccggcggcgaccagactgtacatggtcacgcactggataccacgctgaatgggggataccagtatgtgcacaacggcggtacagcgtctgacactgttgtgaacagtgacggctggcagattgtcaaaaacgggggtgtggccgggaataccaccgttaatcagaagggcagactgcaggtggacgccggtggtacagccacgaatgtcaccctgaagcagggcggcgcactggttaccagtacggctgcaaccgttaccggcataaaccgcctgggagcattctctgttgtggagggtaaagctgataatgtcgtactggaaaatggcggacgcctggatgtgctgaccggacacacagccactaatacccgcgtggatgatggcggaacgctggatgtccgcaacggtggcaccgccaccaccgtatccatgggaaatggcggtgtactgctggccgattccggtgccgctgtcagtggtacccggagcgacggaaaggcattcagtatcggaggcggtcaggcggatgccctgatgctggaaaaaggcagttcattcacgctgaacgccggtgatacggccacggataccacggtaaatggcggactgttcaccgccaggggcggcacactggcgggcaccaccacgctgaataacggcgccaaaggttaaacacccaagcagacgccgcaatatcagcaccaacagaaaggttaaatgacgttgtcggacttctactggcagcaccagaagatagagcgacaggcaagtagcaat

SEQ ID NO: 32 - DNA, 1863 bp, Artificial Sequence
  Synthetic reporter polynucleotide
  misc_feature (1)..(1): 5' Biotinylation
attgcuacttgcctgtcgctctatcttctggtgctgtagtttggatgaccaaggatagccttaacctacttgcctgtcgctctatcttcggcgtctgcttgggtgtttaaccgtctctcttgtccgtgcaatagctcaataatagaataaaacgatcaatatctattttatcgatcgtttatatcgatcgataagctaataataacctttgtcagtaacatgcacagatacgtacagaaagacattcagggaacaacagaaccacaattcagaaactcccacagccggacctccggcactgtaaccctttacctgccggtatccacgtttgtgggtaccggcttttttattcaccctcaatctaaggaaaagctgatgaaacgacatctgaatacctgctacaggctggtatggaatcacatgacgggcgctttcgtggttgcctccgaactggcccgcgcacggggtaaacgtggcggtgtggcggttgcactgtctcttgccgcagtcacgtcactcccggtgctggctgctgacatcgttgtgcacccgggagaaaccgtgaacggcggaacactggcaaatcatgacaaccagattgtcttcggtacgaccaacggaatgaccatcagtaccgggctggagtatgggccggataacgaggccaataccggcgggcaatgggtacaggatggcggaacagccaacaaaacgactgtcaccagtggtggtcttcagagagtgaaccccggtggaagtgtctcagacacggttatcagtgccggaggcggacagagccttcagggacgggctgtgaacaccacgctgaatggtggcgaacagtggatgcatgagggggcgatagccacaggaaccgtcattaatgataagggctggcaggtcgtcaagcccggtacagtggcaacggataccgttgttaataccggggcggaagggggaccggatgcagaaaacggtgataccgggcagtttgttcgcggggatgccgtacgcacaaccatcaataaaaacggtcgccagattgtgagagctgaaggaacggcaaataccactgtggtttatgccggcggcgaccagactgtacatggtcacgcactggataccacgctgaatgggggataccagtatgtgcacaacggcggtacagcgtctgacactgttgtgaacagtgacggctggcagattgtcaaaaacgggggtgtggccgggaataccaccgttaatcagaagggcagactgcaggtggacgccggtggtacagccacgaatgtcaccctgaagcagggcggcgcactggttaccagtacggctgcaaccgttaccggcataaaccgcctgggagcattctctgttgtggagggtaaagctgataatgtcgtactggaaaatggcggacgcctggatgtgctgaccggacacacagccactaatacccgcgtggatgatggcggaacgctggatgtccgcaacggtggcaccgccaccaccgtatccatgggaaatggcggtgtactgctggccgattccggtgccgctgtcagtggtacccggagcgacggaaaggcattcagtatcggaggcggtcaggcggatgccctgatgctggaaaaaggcagttcattcacgctgaacgccggtgatacggccacggataccacggtaaatggcggactgttcaccgccaggggcggcacactggcgggcaccaccacgctgaataacggcgccaaaggttaaacacccaagcagacgccgcaatatcagcaccaacagaaaggttaaggctatccttggtcatccaaactacagcaccagaagatagagcgacaggcaagtagcaat

SEQ ID NO: 33 - DNA, 1077 bp, Artificial Sequence
  Synthetic reporter polynucleotide
  misc_feature (1)..(1): 5' Biotinylation
attgcuacttgcctgtcgctctatcttctaaggttaaaagaaagttgtcggtgtctttgtgcagcacctcactgcctggccgtaaatacgcgtatcaaacggaccaacatcattctggtagtaattaacgtctaactgcggctctgccgagtagctactggtgttctgttcgctgaaaacctggaactgcttggttgaaacggtggcattgaagttttgcaccgcatagccaacgctgaatttttgcgttgcgtagccgtcagtactggaaccgtacttgttatcgaaatcattgaagtagctaggatcgctgaccttggtgtagtcgacgttgaaacgccacacctgatccatgaccccggagtggttccagtagaataaccaacgacgtgaactgtcatcgttcgggtgttcatcttcatagactttatctgaaggcagatagtccagttccatcaagccagcgcccgcctgggagaggtagcggaattcgttctcccacatgatgttgccacgacgatgcatataatgcggcgtgatggtggcatccatatttggcgcgatgttccagtaatatggcaggtagaactcaaagtagttggtggtggtgtacttggcgttcgggatcaagaaaccagagcgacgtttgtcacccaccggcaactgcaaataggggctataaaagatcggtaccggacccaccttaaagcgggcgttccagatctccgcaacttgttcttcgcggtcatgaataatttcgctacctaccacgctccaggtgtcagaacccggcagacaggaggtaaagctaccgttatccagaatggtatagcggttttcgccacgttgtttcatcaggtccgctttaccgcgaccctggcgacccaccatctggtaatcaccttcccagacgttggtatctttggtgttcagattcgcccagcctttcggccctttgaggatcacctggttatcgtcgtaatggacattaccgagcgcatcaacaggtgctgcacaaagacaccgacaactttcttttaaccttgccagcaatatcagcaccaacagaaaagcaat

SEQ ID NO: 34 - DNA, 1077 bp, Artificial Sequence
  Synthetic reporter polynucleotide
  misc_feature (1)..(1): 5' Biotinylation
attgcuacttgcctgtcgctctatcttctaaggttaatcgattccgtttgtagtcgtctgtcagcacctcactgcctggccgtaaatacgcgtatcaaacggaccaacatcattctggtagtaattaacgtctaactgcggctctgccgagtagctactggtgttctgttcgctgaaaacctggaactgcttggttgaaacggtggcattgaagttttgcaccgcatagccaacgctgaatttttgcgttgcgtagccgtcagtactggaaccgtacttgttatcgaaatcattgaagtagctaggatcgctgaccttggtgtagtcgacgttgaaacgccacacctgatccatgaccccggagtggttccagtagaataaccaacgacgtgaactgtcatcgttcgggtgttcatcttcatagactttatctgaaggcagatagtccagttccatcaagccagcgcccgcctgggagaggtagcggaattcgttctcccacatgatgttgccacgacgatgcatataatgcggcgtgatggtggcatccatatttggcgcgatgttccagtaatatggcaggtagaactcaaagtagttggtggtggtgtacttggcgttcgggatcaagaaaccagagcgacgtttgtcacccaccggcaactgcaaataggggctataaaagatcggtaccggacccaccttaaagcgggcgttccagatctccgcaacttgttcttcgcggtcatgaataatttcgctacctaccacgctccaggtgtcagaacccggcagacaggaggtaaagctaccgttatccagaatggtatagcggttttcgccacgttgtttcatcaggtccgctttaccgcgaccctggcgacccaccatctggtaatcaccttcccagacgttggtatctttggtgttcagattcgcccagcctttcggccctttgaggatcacctggttatcgtcgtaatggacattaccgagcgcatcaacaggtgctgacagacgactacaaacggaatcgattaaccttgccagcaatatcagcaccaacagaaaagcaat

SEQ ID NO: 35 - DNA, 1077 bp, Artificial Sequence
  Synthetic reporter polynucleotide
  misc_feature (1)..(1): 5' Biotinylation
attgcuacttgcctgtcgctctatcttctaaggttaagagtcttgtgtcccagttaccaggcagcacctcactgcctggccgtaaatacgcgtatcaaacggaccaacatcattctggtagtaattaacgtctaactgcggctctgccgagtagctactggtgttctgttcgctgaaaacctggaactgcttggttgaaacggtggcattgaagttttgcaccgcatagccaacgctgaatttttgcgttgcgtagccgtcagtactggaaccgtacttgttatcgaaatcattgaagtagctaggatcgctgaccttggtgtagtcgacgttgaaacgccacacctgatccatgaccccggagtggttccagtagaataaccaacgacgtgaactgtcatcgttcgggtgttcatcttcatagactttatctgaaggcagatagtccagttccatcaagccagcgcccgcctgggagaggtagcggaattcgttctcccacatgatgttgccacgacgatgcatataatgcggcgtgatggtggcatccatatttggcgcgatgttccagtaatatggcaggtagaactcaaagtagttggtggtggtgtacttggcgttcgggatcaagaaaccagagcgacgtttgtcacccaccggcaactgcaaataggggctataaaagatcggtaccggacccaccttaaagcgggcgttccagatctccgcaacttgttcttcgcggtcatgaataatttcgctacctaccacgctccaggtgtcagaacccggcagacaggaggtaaagctaccgttatccagaatggtatagcggttttcgccacgttgtttcatcaggtccgctttaccgcgaccctggcgacccaccatctggtaatcaccttcccagacgttggtatctttggtgttcagattcgcccagcctttcggccctttgaggatcacctggttatcgtcgtaatggacattaccgagcgcatcaacaggtgctgcctggtaactgggacacaagactcttaaccttgccagcaatatcagcaccaacagaaaagcaat

SEQ ID NO: 36 - DNA, 1077 bp, Artificial Sequence
  Synthetic reporter polynucleotide
  misc_feature (1)..(1): 5' Biotinylation
attgcuacttgcctgtcgctctatcttctaaggttaattcggattctatcgtgtttccctacagcacctcactgcctggccgtaaatacgcgtatcaaacggaccaacatcattctggtagtaattaacgtctaactgcggctctgccgagtagctactggtgttctgttcgctgaaaacctggaactgcttggttgaaacggtggcattgaagttttgcaccgcatagccaacgctgaatttttgcgttgcgtagccgtcagtactggaaccgtacttgttatcgaaatcattgaagtagctaggatcgctgaccttggtgtagtcgacgttgaaacgccacacctgatccatgaccccggagtggttccagtagaataaccaacgacgtgaactgtcatcgttcgggtgttcatcttcatagactttatctgaaggcagatagtccagttccatcaagccagcgcccgcctgggagaggtagcggaattcgttctcccacatgatgttgccacgacgatgcatataatgcggcgtgatggtggcatccatatttggcgcgatgttccagtaatatggcaggtagaactcaaagtagttggtggtggtgtacttggcgttcgggatcaagaaaccagagcgacgtttgtcacccaccggcaactgcaaataggggctataaaagatcggtaccggacccaccttaaagcgggcgttccagatctccgcaacttgttcttcgcggtcatgaataatttcgctacctaccacgctccaggtgtcagaacccggcagacaggaggtaaagctaccgttatccagaatggtatagcggttttcgccacgttgtttcatcaggtccgctttaccgcgaccctggcgacccaccatctggtaatcaccttcccagacgttggtatctttggtgttcagattcgcccagcctttcggccctttgaggatcacctggttatcgtcgtaatggacattaccgagcgcatcaacaggtgctgtagggaaacacgatagaatccgaattaaccttgccagcaatatcagcaccaacagaaaagcaat

SEQ ID NO: 37 - DNA, 1077 bp, Artificial Sequence
  Synthetic reporter polynucleotide
  misc_feature (1)..(1): 5' Biotinylation
attgcuacttgcctgtcgctctatcttctaaggttaacttgtccagggtttgtgtaaccttcagcacctcactgcctggccgtaaatacgcgtatcaaacggaccaacatcattctggtagtaattaacgtctaactgcggctctgccgagtagctactggtgttctgttcgctgaaaacctggaactgcttggttgaaacggtggcattgaagttttgcaccgcatagccaacgctgaatttttgcgttgcgtagccgtcagtactggaaccgtacttgttatcgaaatcattgaagtagctaggatcgctgaccttggtgtagtcgacgttgaaacgccacacctgatccatgaccccggagtggttccagtagaataaccaacgacgtgaactgtcatcgttcgggtgttcatcttcatagactttatctgaaggcagatagtccagttccatcaagccagcgcccgcctgggagaggtagcggaattcgttctcccacatgatgttgccacgacgatgcatataatgcggcgtgatggtggcatccatatttggcgcgatgttccagtaatatggcaggtagaactcaaagtagttggtggtggtgtacttggcgttcgggatcaagaaaccagagcgacgtttgtcacccaccggcaactgcaaataggggctataaaagatcggtaccggacccaccttaaagcgggcgttccagatctccgcaacttgttcttcgcggtcatgaataatttcgctacctaccacgctccaggtgtcagaacccggcagacaggaggtaaagctaccgttatccagaatggtatagcggttttcgccacgttgtttcatcaggtccgctttaccgcgaccctggcgacccaccatctggtaatcaccttcccagacgttggtatctttggtgttcagattcgcccagcctttcggccctttgaggatcacctggttatcgtcgtaatggacattaccgagcgcatcaacaggtgctgaaggttacacaaaccctggacaagttaaccttgccagcaatatcagcaccaacagaaaagcaat

SEQ ID NO: 38 - DNA, 1077 bp, Artificial Sequence
  Synthetic reporter polynucleotide
  misc_feature (1)..(1): 5' Biotinylation
attgcuacttgcctgtcgctctatcttctaaggttaattctcgcaaaggcagaaagtagtccagcacctcactgcctggccgtaaatacgcgtatcaaacggaccaacatcattctggtagtaattaacgtctaactgcggctctgccgagtagctactggtgttctgttcgctgaaaacctggaactgcttggttgaaacggtggcattgaagttttgcaccgcatagccaacgctgaatttttgcgttgcgtagccgtcagtactggaaccgtacttgttatcgaaatcattgaagtagctaggatcgctgaccttggtgtagtcgacgttgaaacgccacacctgatccatgaccccggagtggttccagtagaataaccaacgacgtgaactgtcatcgttcgggtgttcatcttcatagactttatctgaaggcagatagtccagttccatcaagccagcgcccgcctgggagaggtagcggaattcgttctcccacatgatgttgccacgacgatgcatataatgcggcgtgatggtggcatccatatttggcgcgatgttccagtaatatggcaggtagaactcaaagtagttggtggtggtgtacttggcgttcgggatcaagaaaccagagcgacgtttgtcacccaccggcaactgcaaataggggctataaaagatcggtaccggacccaccttaaagcgggcgttccagatctccgcaacttgttcttcgcggtcatgaataatttcgctacctaccacgctccaggtgtcagaacccggcagacaggaggtaaagctaccgttatccagaatggtatagcggttttcgccacgttgtttcatcaggtccgctttaccgcgaccctggcgacccaccatctggtaatcaccttcccagacgttggtatctttggtgttcagattcgcccagcctttcggccctttgaggatcacctggttatcgtcgtaatggacattaccgagcgcatcaacaggtgctggactactttctgcctttgcgagaattaaccttgccagcaatatcagcaccaacagaaaagcaat

SEQ ID NO: 39 - DNA, 1077 bp, Artificial Sequence
  Synthetic reporter polynucleotide
  misc_feature (1)..(1): 5' Biotinylation
attgcuacttgcctgtcgctctatcttctaaggttaagtgttaccgtgggaatgaatccttcagcacctcactgcctggccgtaaatacgcgtatcaaacggaccaacatcattctggtagtaattaacgtctaactgcggctctgccgagtagctactggtgttctgttcgctgaaaacctggaactgcttggttgaaacggtggcattgaagttttgcaccgcatagccaacgctgaatttttgcgttgcgtagccgtcagtactggaaccgtacttgttatcgaaatcattgaagtagctaggatcgctgaccttggtgtagtcgacgttgaaacgccacacctgatccatgaccccggagtggttccagtagaataaccaacgacgtgaactgtcatcgttcgggtgttcatcttcatagactttatctgaaggcagatagtccagttccatcaagccagcgcccgcctgggagaggtagcggaattcgttctcccacatgatgttgccacgacgatgcatataatgcggcgtgatggtggcatccatatttggcgcgatgttccagtaatatggcaggtagaactcaaagtagttggtggtggtgtacttggcgttcgggatcaagaaaccagagcgacgtttgtcacccaccggcaactgcaaataggggctataaaagatcggtaccggacccaccttaaagcgggcgttccagatctccgcaacttgttcttcgcggtcatgaataatttcgctacctaccacgctccaggtgtcagaacccggcagacaggaggtaaagctaccgttatccagaatggtatagcggttttcgccacgttgtttcatcaggtccgctttaccgcgaccctggcgacccaccatctggtaatcaccttcccagacgttggtatctttggtgttcagattcgcccagcctttcggccctttgaggatcacctggttatcgtcgtaatggacattaccgagcgcatcaacaggtgctgaaggattcattcccacggtaacacttaaccttgccagcaatatcagcaccaacagaaaagcaat

SEQ ID NO: 40 - DNA, 1077 bp, Artificial Sequence
  Synthetic reporter polynucleotide
  misc_feature (1)..(1): 5' Biotinylation
attgcuacttgcctgtcgctctatcttctaaggttaattcagggaacaaaccaagttacgtcagcacctcactgcctggccgtaaatacgcgtatcaaacggaccaacatcattctggtagtaattaacgtctaactgcggctctgccgagtagctactggtgttctgttcgctgaaaacctggaactgcttggttgaaacggtggcattgaagttttgcaccgcatagccaacgctgaatttttgcgttgcgtagccgtcagtactggaaccgtacttgttatcgaaatcattgaagtagctaggatcgctgaccttggtgtagtcgacgttgaaacgccacacctgatccatgaccccggagtggttccagtagaataaccaacgacgtgaactgtcatcgttcgggtgttcatcttcatagactttatctgaaggcagatagtccagttccatcaagccagcgcccgcctgggagaggtagcggaattcgttctcccacatgatgttgccacgacgatgcatataatgcggcgtgatggtggcatccatatttggcgcgatgttccagtaatatggcaggtagaactcaaagtagttggtggtggtgtacttggcgttcgggatcaagaaaccagagcgacgtttgtcacccaccggcaactgcaaataggggctataaaagatcggtaccggacccaccttaaagcgggcgttccagatctccgcaacttgttcttcgcggtcatgaataatttcgctacctaccacgctccaggtgtcagaacccggcagacaggaggtaaagctaccgttatccagaatggtatagcggttttcgccacgttgtttcatcaggtccgctttaccgcgaccctggcgacccaccatctggtaatcaccttcccagacgttggtatctttggtgttcagattcgcccagcctttcggccctttgaggatcacctggttatcgtcgtaatggacattaccgagcgcatcaacaggtgctgacgtaacttggtttgttccctgaattaaccttgccagcaatatcagcaccaacagaaaagcaat

SEQ ID NO: 41 - DNA, 1079 bp, Artificial Sequence
  Synthetic reporter polynucleotide
  misc_feature (1)..(1): 5' Biotinylation
attgcuacttgcctgtcgctctatcttctaaggttaaaagaaagttgtcggtgtctttgtgcagcacctcaatgtaaccgctaccaccggtaaccagaactctcataattcgctccattaggcttatggtatgaaataaccatagcataacaaagatgcgaaaagtgtgacatggaataaattagtggaatcgtttacacaagaatttagccgttttttatgcgcgattaagtgattataaaacagagggtttatgaatgattgcgctttttatctgaaaaaagacgcggtttcatgcctgcatgcgtcgaaccgttggccggagagggtgctaaggccgcctccggcaaggtcagcactaccgactcaatatatttttgtcagcacatagcgatagagtccaccgtccggcacgaactcaagacgatgggtaatacaggcaggcgcatcttcagcgtggtgcgaaacaaacaacaattgcgtttcaccttcgctaatcagcacatcaacaaaacggcggataagctggcgattcagcggatcaagcccctgtagtggttcatcgagaataagcaacgtcggatgtttcaccagtgcgcggacaatcagcgccagacgctgctgtccccaggaaagactatggaacggagcgtcagccgtgcgtttatcaatgccgagaatatccagccactgctgcaccagtttttgctggcgatccgaaacggcctgataaatgccaatcgaatcaaaatagccagaaagaatcacattacgcacggtagtgctgacccggtaatccagatgcaaactactgctgacgtaaccgatatgctttttgatatcccagatggtttcgccgctgccgcgacgtcgtccgaaaagcgtcaaatcgttgctgtaaccttgcggatgatcgccagtaaccaggcttaataacgtcgattttcctgcaccatttggcccgacaatttgccagtgttcgcctggattcacctgccagctaaggtaggtgctgcacaaagacaccgacaactttcttttaaccttgccagcaatatcagcaccaacagaaaagcaat

SEQ ID NO: 42 - DNA, 1079 bp, Artificial Sequence
  Synthetic reporter polynucleotide
  misc_feature (1)..(1): 5' Biotinylation
attgcuacttgcctgtcgctctatcttctaaggttaatcgattccgtttgtagtcgtctgtcagcacctcaatgtaaccgctaccaccggtaaccagaactctcataattcgctccattaggcttatggtatgaaataaccatagcataacaaagatgcgaaaagtgtgacatggaataaattagtggaatcgtttacacaagaatttagccgttttttatgcgcgattaagtgattataaaacagagggtttatgaatgattgcgctttttatctgaaaaaagacgcggtttcatgcctgcatgcgtcgaaccgttggccggagagggtgctaaggccgcctccggcaaggtcagcactaccgactcaatatatttttgtcagcacatagcgatagagtccaccgtccggcacgaactcaagacgatgggtaatacaggcaggcgcatcttcagcgtggtgcgaaacaaacaacaattgcgtttcaccttcgctaatcagcacatcaacaaaacggcggataagctggcgattcagcggatcaagcccctgtagtggttcatcgagaataagcaacgtcggatgtttcaccagtgcgcggacaatcagcgccagacgctgctgtccccaggaaagactatggaacggagcgtcagccgtgcgtttatcaatgccgagaatatccagccactgctgcaccagtttttgctggcgatccgaaacggcctgataaatgccaatcgaatcaaaatagccagaaagaatcacattacgcacggtagtgctgacccggtaatccagatgcaaactactgctgacgtaaccgatatgctttttgatatcccagatggtttcgccgctgccgcgacgtcgtccgaaaagcgtcaaatcgttgctgtaaccttgcggatgatcgccagtaaccaggcttaataacgtcgattttcctgcaccatttggcccgacaatttgccagtgttcgcctggattcacctgccagctaaggtaggtgctgacagacgactacaaacggaatcgattaaccttgccagcaatatcagcaccaacagaaaagcaat

SEQ ID NO: 43 - DNA, 1079 bp, Artificial Sequence
  Synthetic reporter polynucleotide
  misc_feature (1)..(1): 5' Biotinylation
attgcuacttgcctgtcgctctatcttctaaggttaagagtcttgtgtcccagttaccaggcagcacctcaatgtaaccgctaccaccggtaaccagaactctcataattcgctccattaggcttatggtatgaaataaccatagcataacaaagatgcgaaaagtgtgacatggaataaattagtggaatcgtttacacaagaatttagccgttttttatgcgcgattaagtgattataaaacagagggtttatgaatgattgcgctttttatctgaaaaaagacgcggtttcatgcctgcatgcgtcgaaccgttggccggagagggtgctaaggccgcctccggcaaggtcagcactaccgactcaatatatttttgtcagcacatagcgatagagtccaccgtccggcacgaactcaagacgatgggtaatacaggcaggcgcatcttcagcgtggtgcgaaacaaacaacaattgcgtttcaccttcgctaatcagcacatcaacaaaacggcggataagctggcgattcagcggatcaagcccctgtagtggttcatcgagaataagcaacgtcggatgtttcaccagtgcgcggacaatcagcgccagacgctgctgtccccaggaaagactatggaacggagcgtcagccgtgcgtttatcaatgccgagaatatccagccactgctgcaccagtttttgctggcgatccgaaacggcctgataaatgccaatcgaatcaaaatagccagaaagaatcacattacgcacggtagtgctgacccggtaatccagatgcaaactactgctgacgtaaccgatatgctttttgatatcccagatggtttcgccgctgccgcgacgtcgtccgaaaagcgtcaaatcgttgctgtaaccttgcggatgatcgccagtaaccaggcttaataacgtcgattttcctgcaccatttggcccgacaatttgccagtgttcgcctggattcacctgccagctaaggtaggtgctgcctggtaactgggacacaagactcttaaccttgccagcaatatcagcaccaacagaaaagcaat

SEQ ID NO: 44 - DNA, 1079 bp, Artificial Sequence
  Synthetic reporter polynucleotide
  misc_feature (1)..(1): 5' Biotinylation
attgcuacttgcctgtcgctctatcttctaaggttaattcggattctatcgtgtttccctacagcacctcaatgtaaccgctaccaccggtaaccagaactctcataattcgctccattaggcttatggtatgaaataaccatagcataacaaagatgcgaaaagtgtgacatggaataaattagtggaatcgtttacacaagaatttagccgttttttatgcgcgattaagtgattataaaacagagggtttatgaatgattgcgctttttatctgaaaaaagacgcggtttcatgcctgcatgcgtcgaaccgttggccggagagggtgctaaggccgcctccggcaaggtcagcactaccgactcaatatatttttgtcagcacatagcgatagagtccaccgtccggcacgaactcaagacgatgggtaatacaggcaggcgcatcttcagcgtggtgcgaaacaaacaacaattgcgtttcaccttcgctaatcagcacatcaacaaaacggcggataagctggcgattcagcggatcaagcccctgtagtggttcatcgagaataagcaacgtcggatgtttcaccagtgcgcggacaatcagcgccagacgctgctgtccccaggaaagactatggaacggagcgtcagccgtgcgtttatcaatgccgagaatatccagccactgctgcaccagtttttgctggcgatccgaaacggcctgataaatgccaatcgaatcaaaatagccagaaagaatcacattacgcacggtagtgctgacccggtaatccagatgcaaactactgctgacgtaaccgatatgctttttgatatcccagatggtttcgccgctgccgcgacgtcgtccgaaaagcgtcaaatcgttgctgtaaccttgcggatgatcgccagtaaccaggcttaataacgtcgattttcctgcaccatttggcccgacaatttgccagtgttcgcctggattcacctgccagctaaggtaggtgctgtagggaaacacgatagaatccgaattaaccttgccagcaatatcagcaccaacagaaaagcaat

SEQ ID NO: 45 - DNA, 1079 bp, Artificial Sequence
  Synthetic reporter polynucleotide
  misc_feature (1)..(1): 5' Biotinylation
attgcuacttgcctgtcgctctatcttctaaggttaacttgtccagggtttgtgtaaccttcagcacctcaatgtaaccgctaccaccggtaaccagaactctcataattcgctccattaggcttatggtatgaaataaccatagcataacaaagatgcgaaaagtgtgacatggaataaattagtggaatcgtttacacaagaatttagccgttttttatgcgcgattaagtgattataaaacagagggtttatgaatgattgcgctttttatctgaaaaaagacgcggtttcatgcctgcatgcgtcgaaccgttggccggagagggtgctaaggccgcctccggcaaggtcagcactaccgactcaatatatttttgtcagcacatagcgatagagtccaccgtccggcacgaactcaagacgatgggtaatacaggcaggcgcatcttcagcgtggtgcgaaacaaacaacaattgcgtttcaccttcgctaatcagcacatcaacaaaacggcggataagctggcgattcagcggatcaagcccctgtagtggttcatcgagaataagcaacgtcggatgtttcaccagtgcgcggacaatcagcgccagacgctgctgtccccaggaaagactatggaacggagcgtcagccgtgcgtttatcaatgccgagaatatccagccactgctgcaccagtttttgctggcgatccgaaacggcctgataaatgccaatcgaatcaaaatagccagaaagaatcacattacgcacggtagtgctgacccggtaatccagatgcaaactactgctgacgtaaccgatatgctttttgatatcccagatggtttcgccgctgccgcgacgtcgtccgaaaagcgtcaaatcgttgctgtaaccttgcggatgatcgccagtaaccaggcttaataacgtcgattttcctgcaccatttggcccgacaatttgccagtgttcgcctggattcacctgccagctaaggtaggtgctgaaggttacacaaaccctggacaagttaaccttgccagcaatatcagcaccaacagaaaagcaat

SEQ ID NO: 46 - DNA, 1079 bp, Artificial Sequence
  Synthetic reporter polynucleotide
  misc_feature (1)..(1): 5' Biotinylation
attgcuacttgcctgtcgctctatcttctaaggttaattctcgcaaaggcagaaagtagtccagcacctcaatgtaaccgctaccaccggtaaccagaactctcataattcgctccattaggcttatggtatgaaataaccatagcataacaaagatgcgaaaagtgtgacatggaataaattagtggaatcgtttacacaagaatttagccgttttttatgcgcgattaagtgattataaaacagagggtttatgaatgattgcgctttttatctgaaaaaagacgcggtttcatgcctgcatgcgtcgaaccgttggccggagagggtgctaaggccgcctccggcaaggtcagcactaccgactcaatatatttttgtcagcacatagcgatagagtccaccgtccggcacgaactcaagacgatgggtaatacaggcaggcgcatcttcagcgtggtgcgaaacaaacaacaattgcgtttcaccttcgctaatcagcacatcaacaaaacggcggataagctggcgattcagcggatcaagcccctgtagtggttcatcgagaataagcaacgtcggatgtttcaccagtgcgcggacaatcagcgccagacgctgctgtccccaggaaagactatggaacggagcgtcagccgtgcgtttatcaatgccgagaatatccagccactgctgcaccagtttttgctggcgatccgaaacggcctgataaatgccaatcgaatcaaaatagccagaaagaatcacattacgcacggtagtgctgacccggtaatccagatgcaaactactgctgacgtaaccgatatgctttttgatatcccagatggtttcgccgctgccgcgacgtcgtccgaaaagcgtcaaatcgttgctgtaaccttgcggatgatcgccagtaaccaggcttaataacgtcgattttcctgcaccatttggcccgacaatttgccagtgttcgcctggattcacctgccagctaaggtaggtgctggactactttctgcctttgcgagaattaaccttgccagcaatatcagcaccaacagaaaagcaat

SEQ ID NO: 47 - DNA, 1079 bp, Artificial Sequence
  Synthetic reporter polynucleotide
  misc_feature (1)..(1): 5' Biotinylation
attgcuacttgcctgtcgctctatcttctaaggttaagtgttaccgtgggaatgaatccttcagcacctcaatgtaaccgctaccaccggtaaccagaactctcataattcgctccattaggcttatggtatgaaataaccatagcataacaaagatgcgaaaagtgtgacatggaataaattagtggaatcgtttacacaagaatttagccgttttttatgcgcgattaagtgattataaaacagagggtttatgaatgattgcgctttttatctgaaaaaagacgcggtttcatgcctgcatgcgtcgaaccgttggccggagagggtgctaaggccgcctccggcaaggtcagcactaccgactcaatatatttttgtcagcacatagcgatagagtccaccgtccggcacgaactcaagacgatgggtaatacaggcaggcgcatcttcagcgtggtgcgaaacaaacaacaattgcgtttcaccttcgctaatcagcacatcaacaaaacggcggataagctggcgattcagcggatcaagcccctgtagtggttcatcgagaataagcaacgtcggatgtttcaccagtgcgcggacaatcagcgccagacgctgctgtccccaggaaagactatggaacggagcgtcagccgtgcgtttatcaatgccgagaatatccagccactgctgcaccagtttttgctggcgatccgaaacggcctgataaatgccaatcgaatcaaaatagccagaaagaatcacattacgcacggtagtgctgacccggtaatccagatgcaaactactgctgacgtaaccgatatgctttttgatatcccagatggtttcgccgctgccgcgacgtcgtccgaaaagcgtcaaatcgttgctgtaaccttgcggatgatcgccagtaaccaggcttaataacgtcgattttcctgcaccatttggcccgacaatttgccagtgttcgcctggattcacctgccagctaaggtaggtgctgaaggattcattcccacggtaacacttaaccttgccagcaatatcagcaccaacagaaaagcaat

SEQ ID NO: 48 - DNA, 1079 bp, Artificial Sequence
  Synthetic reporter polynucleotide
  misc_feature (1)..(1): 5' Biotinylation
attgcuacttgcctgtcgctctatcttctaaggttaattcagggaacaaaccaagttacgtcagcacctcaatgtaaccgctaccaccggtaaccagaactctcataattcgctccattaggcttatggtatgaaataaccatagcataacaaagatgcgaaaagtgtgacatggaataaattagtggaatcgtttacacaagaatttagccgttttttatgcgcgattaagtgattataaaacagagggtttatgaatgattgcgctttttatctgaaaaaagacgcggtttcatgcctgcatgcgtcgaaccgttggccggagagggtgctaaggccgcctccggcaaggtcagcactaccgactcaatatatttttgtcagcacatagcgatagagtccaccgtccggcacgaactcaagacgatgggtaatacaggcaggcgcatcttcagcgtggtgcgaaacaaacaacaattgcgtttcaccttcgctaatcagcacatcaacaaaacggcggataagctggcgattcagcggatcaagcccctgtagtggttcatcgagaataagcaacgtcggatgtttcaccagtgcgcggacaatcagcgccagacgctgctgtccccaggaaagactatggaacggagcgtcagccgtgcgtttatcaatgccgagaatatccagccactgctgcaccagtttttgctggcgatccgaaacggcctgataaatgccaatcgaatcaaaatagccagaaagaatcacattacgcacggtagtgctgacccggtaatccagatgcaaactactgctgacgtaaccgatatgctttttgatatcccagatggtttcgccgctgccgcgacgtcgtccgaaaagcgtcaaatcgttgctgtaaccttgcggatgatcgccagtaaccaggcttaataacgtcgattttcctgcaccatttggcccgacaatttgccagtgttcgcctggattcacctgccagctaaggtaggtgctgacgtaacttggtttgttccctgaattaaccttgccagcaatatcagcaccaacagaaaagcaat

SEQ ID NO: 49 - DNA, 1077 bp, Artificial Sequence
  Synthetic reporter polynucleotide
  misc_feature (1)..(1): 5' Biotinylation
attgcuacttgcctgtcgctctatcttctaaggttaaaagaaagttgtcggtgtctttgtgcagcacctaattaaacccggctaccccacaaatcgtactcatcggcgtgctcgactttcacacgcaggatatcacccggcttaacgttggtttcaccattgagataaaccgcgccgtcgatttccggtgcatctgccatgctgcgaccaatcgcgccttcttcgtccacttcgtcgataatcaccagaatttcacggcccactttctcttgcaggcgctcggcggaaatctgctgctgcagctgcatgaaacggttccagcgttcttctttaacttcttccggaacctggtcaggcagggcattggcgtctgcaccttcaaccgggctgtatttaaagcagccaacgcgatccagacgcgcttctttcaggaagtcgagtagcatctggaaatcttcttctgtctcgccagggaagccgacaataaaggttgagcgtagggtcagttccgggcagatttcgcgccactgtttgatgcgcgccagttggcgatctacagaacccggacgcttcatcagtttgagaatgcgcgggctggcgtgctgcaacggaatgtccagatacggcaggattttgccttctgccatcagtgggatgacgtcgtccacatgcggataagggtaaacgtagtgcagacgtgtccagatccccagtttcgataactgttcgcacaggctgaccatgctggtttttaccggctcgccgttgtggaagccagtacgatgtttaacatcaacgccataggcggaagtatcctgcgagatcaccagaatctctttaacgcccgcatctaccagacgtttcgcttcacttaacacttcgccaatcggacggctcaccaggtcgccgcgcatagacggaataatgcagaaggtgcagcggtgattacagccttcagaaattttcagataggcataatgacgcggcgtcagtttcacaccttgtaggtgctgcacaaagacaccgacaactttcttttaaccttgccagcaatatcagcaccaacagaaaagcaat

SEQ ID NO: 50 - DNA, 1077 bp, Artificial Sequence
  Synthetic reporter polynucleotide
  misc_feature (1)..(1): 5' Biotinylation
attgcuacttgcctgtcgctctatcttctaaggttaatcgattccgtttgtagtcgtctgtcagcacctaattaaacccggctaccccacaaatcgtactcatcggcgtgctcgactttcacacgcaggatatcacccggcttaacgttggtttcaccattgagataaaccgcgccgtcgatttccggtgcatctgccatgctgcgaccaatcgcgccttcttcgtccacttcgtcgataatcaccagaatttcacggcccactttctcttgcaggcgctcggcggaaatctgctgctgcagctgcatgaaacggttccagcgttcttctttaacttcttccggaacctggtcaggcagggcattggcgtctgcaccttcaaccgggctgtatttaaagcagccaacgcgatccagacgcgcttctttcaggaagtcgagtagcatctggaaatcttcttctgtctcgccagggaagccgacaataaaggttgagcgtagggtcagttccgggcagatttcgcgccactgtttgatgcgcgccagttggcgatctacagaacccggacgcttcatcagtttgagaatgcgcgggctggcgtgctgcaacggaatgtccagatacggcaggattttgccttctgccatcagtgggatgacgtcgtccacatgcggataagggtaaacgtagtgcagacgtgtccagatccccagtttcgataactgttcgcacaggctgaccatgctggtttttaccggctcgccgttgtggaagccagtacgatgtttaacatcaacgccataggcggaagtatcctgcgagatcaccagaatctctttaacgcccgcatctaccagacgtttcgcttcacttaacacttcgccaatcggacggctcaccaggtcgccgcgcatagacggaataatgcagaaggtgcagcggtgattacagccttcagaaattttcagataggcataatgacgcggcgtcagtttcacaccttgtaggtgctgacagacgactacaaacggaatcgattaaccttgccagcaatatcagcaccaacagaaaagcaat

SEQ ID NO: 51 - DNA, 1077 bp, Artificial Sequence
  Synthetic reporter polynucleotide
  misc_feature (1)..(1): 5' Biotinylation
attgcuacttgcctgtcgctctatcttctaaggttaagagtcttgtgtcccagttaccaggcagcacctaattaaacccggctaccccacaaatcgtactcatcggcgtgctcgactttcacacgcaggatatcacccggcttaacgttggtttcaccattgagataaaccgcgccgtcgatttccggtgcatctgccatgctgcgaccaatcgcgccttcttcgtccacttcgtcgataatcaccagaatttcacggcccactttctcttgcaggcgctcggcggaaatctgctgctgcagctgcatgaaacggttccagcgttcttctttaacttcttccggaacctggtcaggcagggcattggcgtctgcaccttcaaccgggctgtatttaaagcagccaacgcgatccagacgcgcttctttcaggaagtcgagtagcatctggaaatcttcttctgtctcgccagggaagccgacaataaaggttgagcgtagggtcagttccgggcagatttcgcgccactgtttgatgcgcgccagttggcgatctacagaacccggacgcttcatcagtttgagaatgcgcgggctggcgtgctgcaacggaatgtccagatacggcaggattttgccttctgccatcagtgggatgacgtcgtccacatgcggataagggtaaacgtagtgcagacgtgtccagatccccagtttcgataactgttcgcacaggctgaccatgctggtttttaccggctcgccgttgtggaagccagtacgatgtttaacatcaacgccataggcggaagtatcctgcgagatcaccagaatctctttaacgcccgcatctaccagacgtttcgcttcacttaacacttcgccaatcggacggctcaccaggtcgccgcgcatagacggaataatgcagaaggtgcagcggtgattacagccttcagaaattttcagataggcataatgacgcggcgtcagtttcacaccttgtaggtgctgcctggtaactgggacacaagactcttaaccttgccagcaatatcagcaccaacagaaaagcaat

SEQ ID NO: 52 - DNA, 1077 bp, Artificial Sequence
  Synthetic reporter polynucleotide
  misc_feature (1)..(1): 5' Biotinylation
attgcuacttgcctgtcgctctatcttctaaggttaattcggattctatcgtgtttccctacagcacctaattaaacccggctaccccacaaatcgtactcatcggcgtgctcgactttcacacgcaggatatcacccggcttaacgttggtttcaccattgagataaaccgcgccgtcgatttccggtgcatctgccatgctgcgaccaatcgcgccttcttcgtccacttcgtcgataatcaccagaatttcacggcccactttctcttgcaggcgctcggcggaaatctgctgctgcagctgcatgaaacggttccagcgttcttctttaacttcttccggaacctggtcaggcagggcattggcgtctgcaccttcaaccgggctgtatttaaagcagccaacgcgatccagacgcgcttctttcaggaagtcgagtagcatctggaaatcttcttctgtctcgccagggaagccgacaataaaggttgagcgtagggtcagttccgggcagatttcgcgccactgtttgatgcgcgccagttggcgatctacagaacccggacgcttcatcagtttgagaatgcgcgggctggcgtgctgcaacggaatgtccagatacggcaggattttgccttctgccatcagtgggatgacgtcgtccacatgcggataagggtaaacgtagtgcagacgtgtccagatccccagtttcgataactgttcgcacaggctgaccatgctggtttttaccggctcgccgttgtggaagccagtacgatgtttaacatcaacgccataggcggaagtatcctgcgagatcaccagaatctctttaacgcccgcatctaccagacgtttcgcttcacttaacacttcgccaatcggacggctcaccaggtcgccgcgcatagacggaataatgcagaaggtgcagcggtgattacagccttcagaaattttcagataggcataatgacgcggcgtcagtttcacaccttgtaggtgctgtagggaaacacgatagaatccgaattaaccttgccagcaatatcagcaccaacagaaaagcaat

SEQ ID NO: 53 - DNA, 1077 bp, Artificial Sequence
  Synthetic reporter polynucleotide
  misc_feature (1)..(1): 5' Biotinylation
attgcuacttgcctgtcgctctatcttctaaggttaacttgtccagggtttgtgtaaccttcagcacctaattaaacccggctaccccacaaatcgtactcatcggcgtgctcgactttcacacgcaggatatcacccggcttaacgttggtttcaccattgagataaaccgcgccgtcgatttccggtgcatctgccatgctgcgaccaatcgcgccttcttcgtccacttcgtcgataatcaccagaatttcacggcccactttctcttgcaggcgctcggcggaaatctgctgctgcagctgcatgaaacggttccagcgttcttctttaacttcttccggaacctggtcaggcagggcattggcgtctgcaccttcaaccgggctgtatttaaagcagccaacgcgatccagacgcgcttctttcaggaagtcgagtagcatctggaaatcttcttctgtctcgccagggaagccgacaataaaggttgagcgtagggtcagttccgggcagatttcgcgccactgtttgatgcgcgccagttggcgatctacagaacccggacgcttcatcagtttgagaatgcgcgggctggcgtgctgcaacggaatgtccagatacggcaggattttgccttctgccatcagtgggatgacgtcgtccacatgcggataagggtaaacgtagtgcagacgtgtccagatccccagtttcgataactgttcgcacaggctgaccatgctggtttttaccggctcgccgttgtggaagccagtacgatgtttaacatcaacgccataggcggaagtatcctgcgagatcaccagaatctctttaacgcccgcatctaccagacgtttcgcttcacttaacacttcgccaatcggacggctcaccaggtcgccgcgcatagacggaataatgcagaaggtgcagcggtgattacagccttcagaaattttcagataggcataatgacgcggcgtcagtttcacaccttgtaggtgctgaaggttacacaaaccctggacaagttaaccttgccagcaatatcagcaccaacagaaaagcaat

SEQ ID NO: 54 - DNA, 1077 bp, Artificial Sequence
  Synthetic reporter polynucleotide
  misc_feature (1)..(1): 5' Biotinylation
attgcuacttgcctgtcgctctatcttctaaggttaattctcgcaaaggcagaaagtagtccagcacctaattaaacccggctaccccacaaatcgtactcatcggcgtgctcgactttcacacgcaggatatcacccggcttaacgttggtttcaccattgagataaaccgcgccgtcgatttccggtgcatctgccatgctgcgaccaatcgcgccttcttcgtccacttcgtcgataatcaccagaatttcacggcccactttctcttgcaggcgctcggcggaaatctgctgctgcagctgcatgaaacggttccagcgttcttctttaacttcttccggaacctggtcaggcagggcattggcgtctgcaccttcaaccgggctgtatttaaagcagccaacgcgatccagacgcgcttctttcaggaagtcgagtagcatctggaaatcttcttctgtctcgccagggaagccgacaataaaggttgagcgtagggtcagttccgggcagatttcgcgccactgtttgatgcgcgccagttggcgatctacagaacccggacgcttcatcagtttgagaatgcgcgggctggcgtgctgcaacggaatgtccagatacggcaggattttgccttctgccatcagtgggatgacgtcgtccacatgcggataagggtaaacgtagtgcagacgtgtccagatccccagtttcgataactgttcgcacaggctgaccatgctggtttttaccggctcgccgttgtggaagccagtacgatgtttaacatcaacgccataggcggaagtatcctgcgagatcaccagaatctctttaacgcccgcatctaccagacgtttcgcttcacttaacacttcgccaatcggacggctcaccaggtcgccgcgcatagacggaataatgcagaaggtgcagcggtgattacagccttcagaaattttcagataggcataatgacgcggcgtcagtttcacaccttgtaggtgctggactactttctgcctttgcgagaattaaccttgccagcaatatcagcaccaacagaaaagcaat

SEQ ID NO: 55 - DNA, 1077 bp, Artificial Sequence
  Synthetic reporter polynucleotide
  misc_feature (1)..(1): 5' Biotinylation
attgcuacttgcctgtcgctctatcttctaaggttaagtgttaccgtgggaatgaatccttcagcacctaattaaacccggctaccccacaaatcgtactcatcggcgtgctcgactttcacacgcaggatatcacccggcttaacgttggtttcaccattgagataaaccgcgccgtcgatttccggtgcatctgccatgctgcgaccaatcgcgccttcttcgtccacttcgtcgataatcaccagaatttcacggcccactttctcttgcaggcgctcggcggaaatctgctgctgcagctgcatgaaacggttccagcgttcttctttaacttcttccggaacctggtcaggcagggcattggcgtctgcaccttcaaccgggctgtatttaaagcagccaacgcgatccagacgcgcttctttcaggaagtcgagtagcatctggaaatcttcttctgtctcgccagggaagccgacaataaaggttgagcgtagggtcagttccgggcagatttcgcgccactgtttgatgcgcgccagttggcgatctacagaacccggacgcttcatcagtttgagaatgcgcgggctggcgtgctgcaacggaatgtccagatacggcaggattttgccttctgccatcagtgggatgacgtcgtccacatgcggataagggtaaacgtagtgcagacgtgtccagatccccagtttcgataactgttcgcacaggctgaccatgctggtttttaccggctcgccgttgtggaagccagtacgatgtttaacatcaacgccataggcggaagtatcctgcgagatcaccagaatctctttaacgcccgcatctaccagacgtttcgcttcacttaacacttcgccaatcggacggctcaccaggtcgccgcgcatagacggaataatgcagaaggtgcagcggtgattacagccttcagaaattttcagataggcataatgacgcggcgtcagtttcacaccttgtaggtgctgaaggattcattcccacggtaacacttaaccttgccagcaatatcagcaccaacagaaaagcaat

SEQ ID NO: 56 - DNA, 1077 bp, Artificial Sequence
  Synthetic reporter polynucleotide
  misc_feature (1)..(1): 5' Biotinylation
attgcuacttgcctgtcgctctatcttctaaggttaattcagggaacaaaccaagttacgtcagcacctaattaaacccggctaccccacaaatcgtactcatcggcgtgctcgactttcacacgcaggatatcacccggcttaacgttggtttcaccattgagataaaccgcgccgtcgatttccggtgcatctgccatgctgcgaccaatcgcgccttcttcgtccacttcgtcgataatcaccagaatttcacggcccactttctcttgcaggcgctcggcggaaatctgctgctgcagctgcatgaaacggttccagcgttcttctttaacttcttccggaacctggtcaggcagggcattggcgtctgcaccttcaaccgggctgtatttaaagcagccaacgcgatccagacgcgcttctttcaggaagtcgagtagcatctggaaatcttcttctgtctcgccagggaagccgacaataaaggttgagcgtagggtcagttccgggcagatttcgcgccactgtttgatgcgcgccagttggcgatctacagaacccggacgcttcatcagtttgagaatgcgcgggctggcgtgctgcaacggaatgtccagatacggcaggattttgccttctgccatcagtgggatgacgtcgtccacatgcggataagggtaaacgtagtgcagacgtgtccagatccccagtttcgataactgttcgcacaggctgaccatgctggtttttaccggctcgccgttgtggaagccagtacgatgtttaacatcaacgccataggcggaagtatcctgcgagatcaccagaatctctttaacgcccgcatctaccagacgtttcgcttcacttaacacttcgccaatcggacggctcaccaggtcgccgcgcatagacggaataatgcagaaggtgcagcggtgattacagccttcagaaattttcagataggcataatgacgcggcgtcagtttcacaccttgtaggtgctgacgtaacttggtttgttccctgaattaaccttgccagcaatatcagcaccaacagaaaagcaat

SEQ ID NO: 57 - DNA, 1078 bp, Artificial Sequence
  Synthetic reporter polynucleotide
  misc_feature (1)..(1): 5' Biotinylation
attgcuacttgcctgtcgctctatcttctaaggttaaaagaaagttgtcggtgtctttgtgcagcacctgatggtgaccggcattcttccgctgttgattagcctgctggttatcatgaacgcactgattaattttatcggtcagcatcgtattgaacgttttgctcaacgttgcgccggtaaccctgtttcccgttacctactgttaccgtgcattggcacgtttgtcttttgcaatccgatgaccctaagcctgggtcgctttatgccggaaaagtacaaacccagctactacgcggcggcctcttatagctgccactcaatgaatggcctcttcccccatatcaaccctggcgaactgtttgtttatcttggcattgccagcggtctgacaacgctgaacctgccacttggcccactggcggtgagttatctgctggttggtctggtcaccaatttcttccgcggctgggtgaccgatctgaccaccgccatttttgagaaaaagatgggcattcaacttgaacaaaaagttcacctggcaggagcaacatcatgacgcatattcggatcgaaaaaggaacgggtggctggggcggcccgcttgagctgaaagccacgccgggaaaaaaaatcgtctatatcaccgccggtacccggcctgcgattgttgacaaactggcacagcttactggctggcaggctattgacggatttaaagaaggtgaacccgcggaggcggaaattggtgtcgcggtaatcgactgtggcggcacattacgctgcggcatctatccgaaacgacgtattcccaccattaatatccactcgacgggcaagtccggtccgctggcgcagtacattgtggaagatatttatgtctctggcgtaaaagaagaaaacatcactgtagtaggtgatgcgacaccacaaccctcttccgtgggccgtgactatgacaccagtaagaaaatcaccgaacaaagcgatggtttactggcgaaggaggtgctgcacaaagacaccgacaactttcttttaaccttgccagcaatatcagcaccaacagaaaagcaat

SEQ ID NO: 58 - DNA, 1078 bp, Artificial Sequence
  Synthetic reporter polynucleotide
  misc_feature (1)..(1): 5' Biotinylation
attgcuacttgcctgtcgctctatcttctaaggttaatcgattccgtttgtagtcgtctgtcagcacctgatggtgaccggcattcttccgctgttgattagcctgctggttatcatgaacgcactgattaattttatcggtcagcatcgtattgaacgttttgctcaacgttgcgccggtaaccctgtttcccgttacctactgttaccgtgcattggcacgtttgtcttttgcaatccgatgaccctaagcctgggtcgctttatgccggaaaagtacaaacccagctactacgcggcggcctcttatagctgccactcaatgaatggcctcttcccccatatcaaccctggcgaactgtttgtttatcttggcattgccagcggtctgacaacgctgaacctgccacttggcccactggcggtgagttatctgctggttggtctggtcaccaatttcttccgcggctgggtgaccgatctgaccaccgccatttttgagaaaaagatgggcattcaacttgaacaaaaagttcacctggcaggagcaacatcatgacgcatattcggatcgaaaaaggaacgggtggctggggcggcccgcttgagctgaaagccacgccgggaaaaaaaatcgtctatatcaccgccggtacccggcctgcgattgttgacaaactggcacagcttactggctggcaggctattgacggatttaaagaaggtgaacccgcggaggcggaaattggtgtcgcggtaatcgactgtggcggcacattacgctgcggcatctatccgaaacgacgtattcccaccattaatatccactcgacgggcaagtccggtccgctggcgcagtacattgtggaagatatttatgtctctggcgtaaaagaagaaaacatcactgtagtaggtgatgcgacaccacaaccctcttccgtgggccgtgactatgacaccagtaagaaaatcaccgaacaaagcgatggtttactggcgaaggaggtgctgacagacgactacaaacggaatcgattaaccttgccagcaatatcagcaccaacagaaaagcaat

SEQ ID NO: 59 - DNA, 1078 bp, Artificial Sequence
  Synthetic reporter polynucleotide
  misc_feature (1)..(1): 5' Biotinylation
attgcuacttgcctgtcgctctatcttctaaggttaagagtcttgtgtcccagttaccaggcagcacctgatggtgaccggcattcttccgctgttgattagcctgctggttatcatgaacgcactgattaattttatcggtcagcatcgtattgaacgttttgctcaacgttgcgccggtaaccctgtttcccgttacctactgttaccgtgcattggcacgtttgtcttttgcaatccgatgaccctaagcctgggtcgctttatgccggaaaagtacaaacccagctactacgcggcggcctcttatagctgccactcaatgaatggcctcttcccccatatcaaccctggcgaactgtttgtttatcttggcattgccagcggtctgacaacgctgaacctgccacttggcccactggcggtgagttatctgctggttggtctggtcaccaatttcttccgcggctgggtgaccgatctgaccaccgccatttttgagaaaaagatgggcattcaacttgaacaaaaagttcacctggcaggagcaacatcatgacgcatattcggatcgaaaaaggaacgggtggctggggcggcccgcttgagctgaaagccacgccgggaaaaaaaatcgtctatatcaccgccggtacccggcctgcgattgttgacaaactggcacagcttactggctggcaggctattgacggatttaaagaaggtgaacccgcggaggcggaaattggtgtcgcggtaatcgactgtggcggcacattacgctgcggcatctatccgaaacgacgtattcccaccattaatatccactcgacgggcaagtccggtccgctggcgcagtacattgtggaagatatttatgtctctggcgtaaaagaagaaaacatcactgtagtaggtgatgcgacaccacaaccctcttccgtgggccgtgactatgacaccagtaagaaaatcaccgaacaaagcgatggtttactggcgaaggaggtgctgcctggtaactgggacacaagactcttaaccttgccagcaatatcagcaccaacagaaaagcaat

SEQ ID NO: 60 - DNA, 1078 bp, Artificial Sequence
  Synthetic reporter polynucleotide
  misc_feature (1)..(1): 5' Biotinylation
attgcuacttgcctgtcgctctatcttctaaggttaattcggattctatcgtgtttccctacagcacctgatggtgaccggcattcttccgctgttgattagcctgctggttatcatgaacgcactgattaattttatcggtcagcatcgtattgaacgttttgctcaacgttgcgccggtaaccctgtttcccgttacctactgttaccgtgcattggcacgtttgtcttttgcaatccgatgaccctaagcctgggtcgctttatgccggaaaagtacaaacccagctactacgcggcggcctcttatagctgccactcaatgaatggcctcttcccccatatcaaccctggcgaactgtttgtttatcttggcattgccagcggtctgacaacgctgaacctgccacttggcccactggcggtgagttatctgctggttggtctggtcaccaatttcttccgcggctgggtgaccgatctgaccaccgccatttttgagaaaaagatgggcattcaacttgaacaaaaagttcacctggcaggagcaacatcatgacgcatattcggatcgaaaaaggaacgggtggctggggcggcccgcttgagctgaaagccacgccgggaaaaaaaatcgtctatatcaccgccggtacccggcctgcgattgttgacaaactggcacagcttactggctggcaggctattgacggatttaaagaaggtgaacccgcggaggcggaaattggtgtcgcggtaatcgactgtggcggcacattacgctgcggcatctatccgaaacgacgtattcccaccattaatatccactcgacgggcaagtccggtccgctggcgcagtacattgtggaagatatttatgtctctggcgtaaaagaagaaaacatcactgtagtaggtgatgcgacaccacaaccctcttccgtgggccgtgactatgacaccagtaagaaaatcaccgaacaaagcgatggtttactggcgaaggaggtgctgtagggaaacacgatagaatccgaattaaccttgccagcaatatcagcaccaacagaaaagcaat

SEQ ID NO: 61 - DNA, 1078 bp, Artificial Sequence
  Synthetic reporter polynucleotide
  misc_feature (1)..(1): 5' Biotinylation
attgcuacttgcctgtcgctctatcttctaaggttaacttgtccagggtttgtgtaaccttcagcacctgatggtgaccggcattcttccgctgttgattagcctgctggttatcatgaacgcactgattaattttatcggtcagcatcgtattgaacgttttgctcaacgttgcgccggtaaccctgtttcccgttacctactgttaccgtgcattggcacgtttgtcttttgcaatccgatgaccctaagcctgggtcgctttatgccggaaaagtacaaacccagctactacgcggcggcctcttatagctgccactcaatgaatggcctcttcccccatatcaaccctggcgaactgtttgtttatcttggcattgccagcggtctgacaacgctgaacctgccacttggcccactggcggtgagttatctgctggttggtctggtcaccaatttcttccgcggctgggtgaccgatctgaccaccgccatttttgagaaaaagatgggcattcaacttgaacaaaaagttcacctggcaggagcaacatcatgacgcatattcggatcgaaaaaggaacgggtggctggggcggcccgcttgagctgaaagccacgccgggaaaaaaaatcgtctatatcaccgccggtacccggcctgcgattgttgacaaactggcacagcttactggctggcaggctattgacggatttaaagaaggtgaacccgcggaggcggaaattggtgtcgcggtaatcgactgtggcggcacattacgctgcggcatctatccgaaacgacgtattcccaccattaatatccactcgacgggcaagtccggtccgctggcgcagtacattgtggaagatatttatgtctctggcgtaaaagaagaaaacatcactgtagtaggtgatgcgacaccacaaccctcttccgtgggccgtgactatgacaccagtaagaaaatcaccgaacaaagcgatggtttactggcgaaggaggtgctgaaggttacacaaaccctggacaagttaaccttgccagcaatatcagcaccaacagaaaagcaat

SEQ ID NO: 62 - DNA, 1078 bp, Artificial Sequence
  Synthetic reporter polynucleotide
  misc_feature (1)..(1): 5' Biotinylation
attgcuacttgcctgtcgctctatcttctaaggttaattctcgcaaaggcagaaagtagtccagcacctgatggtgaccggcattcttccgctgttgattagcctgctggttatcatgaacgcactgattaattttatcggtcagcatcgtattgaacgttttgctcaacgttgcgccggtaaccctgtttcccgttacctactgttaccgtgcattggcacgtttgtcttttgcaatccgatgaccctaagcctgggtcgctttatgccggaaaagtacaaacccagctactacgcggcggcctcttatagctgccactcaatgaatggcctcttcccccatatcaaccctggcgaactgtttgtttatcttggcattgccagcggtctgacaacgctgaacctgccacttggcccactggcggtgagttatctgctggttggtctggtcaccaatttcttccgcggctgggtgaccgatctgaccaccgccatttttgagaaaaagatgggcattcaacttgaacaaaaagttcacctggcaggagcaacatcatgacgcatattcggatcgaaaaaggaacgggtggctggggcggcccgcttgagctgaaagccacgccgggaaaaaaaatcgtctatatcaccgccggtacccggcctgcgattgttgacaaactggcacagcttactggctggcaggctattgacggatttaaagaaggtgaacccgcggaggcggaaattggtgtcgcggtaatcgactgtggcggcacattacgctgcggcatctatccgaaacgacgtattcccaccattaatatccactcgacgggcaagtccggtccgctggcgcagtacattgtggaagatatttatgtctctggcgtaaaagaagaaaacatcactgtagtaggtgatgcgacaccacaaccctcttccgtgggccgtgactatgacaccagtaagaaaatcaccgaacaaagcgatggtttactggcgaaggaggtgctggactactttctgcctttgcgagaattaaccttgccagcaatatcagcaccaacagaaaagcaat

SEQ ID NO: 63 - DNA, 1078 bp, Artificial Sequence
  Synthetic reporter polynucleotide
  misc_feature (1)..(1): 5' Biotinylation
attgcuacttgcctgtcgctctatcttctaaggttaagtgttaccgtgggaatgaatccttcagcacctgatggtgaccggcattcttccgctgttgattagcctgctggttatcatgaacgcactgattaattttatcggtcagcatcgtattgaacgttttgctcaacgttgcgccggtaaccctgtttcccgttacctactgttaccgtgcattggcacgtttgtcttttgcaatccgatgaccctaagcctgggtcgctttatgccggaaaagtacaaacccagctactacgcggcggcctcttatagctgccactcaatgaatggcctcttcccccatatcaaccctggcgaactgtttgtttatcttggcattgccagcggtctgacaacgctgaacctgccacttggcccactggcggtgagttatctgctggttggtctggtcaccaatttcttccgcggctgggtgaccgatctgaccaccgccatttttgagaaaaagatgggcattcaacttgaacaaaaagttcacctggcaggagcaacatcatgacgcatattcggatcgaaaaaggaacgggtggctggggcggcccgcttgagctgaaagccacgccgggaaaaaaaatcgtctatatcaccgccggtacccggcctgcgattgttgacaaactggcacagcttactggctggcaggctattgacggatttaaagaaggtgaacccgcggaggcggaaattggtgtcgcggtaatcgactgtggcggcacattacgctgcggcatctatccgaaacgacgtattcccaccattaatatccactcgacgggcaagtccggtccgctggcgcagtacattgtggaagatatttatgtctctggcgtaaaagaagaaaacatcactgtagtaggtgatgcgacaccacaaccctcttccgtgggccgtgactatgacaccagtaagaaaatcaccgaacaaagcgatggtttactggcgaaggaggtgctgaaggattcattcccacggtaacacttaaccttgccagcaatatcagcaccaacagaaaagcaat

SEQ ID NO: 64 - DNA, 1078 bp, Artificial Sequence
  Synthetic reporter polynucleotide
  misc_feature (1)..(1): 5' Biotinylation
attgcuacttgcctgtcgctctatcttctaaggttaattcagggaacaaaccaagttacgtcagcacctgatggtgaccggcattcttccgctgttgattagcctgctggttatcatgaacgcactgattaattttatcggtcagcatcgtattgaacgttttgctcaacgttgcgccggtaaccctgtttcccgttacctactgttaccgtgcattggcacgtttgtcttttgcaatccgatgaccctaagcctgggtcgctttatgccggaaaagtacaaacccagctactacgcggcggcctcttatagctgccactcaatgaatggcctcttcccccatatcaaccctggcgaactgtttgtttatcttggcattgccagcggtctgacaacgctgaacctgccacttggcccactggcggtgagttatctgctggttggtctggtcaccaatttcttccgcggctgggtgaccgatctgaccaccgccatttttgagaaaaagatgggcattcaacttgaacaaaaagttcacctggcaggagcaacatcatgacgcatattcggatcgaaaaaggaacgggtggctggggcggcccgcttgagctgaaagccacgccgggaaaaaaaatcgtctatatcaccgccggtacccggcctgcgattgttgacaaactggcacagcttactggctggcaggctattgacggatttaaagaaggtgaacccgcggaggcggaaattggtgtcgcggtaatcgactgtggcggcacattacgctgcggcatctatccgaaacgacgtattcccaccattaatatccactcgacgggcaagtccggtccgctggcgcagtacattgtggaagatatttatgtctctggcgtaaaagaagaaaacatcactgtagtaggtgatgcgacaccacaaccctcttccgtgggccgtgactatgacaccagtaagaaaatcaccgaacaaagcgatggtttactggcgaaggaggtgctgacgtaacttggtttgttccctgaattaaccttgccagcaatatcagcaccaacagaaaagcaat